European Patent Application EP 4 137 566 A1, published February 22, 2023. Title: Method for selecting organelle transformant. Applicant: NATIONAL UNIVERSITY CORPORATION KOBE UNIVERSITY. The sequence listing filed with the application follows.

SEQUENCE LISTING (17 sequences)

SEQ ID NO: 1 - DNA, 6753 bp, Saccharomyces cerevisiae
  CDS (1)..(6753)
atgactattcatctattgtattttcatgcaaatagggggcaagaaaacatgagcgaagaaagcttattcgagtcttctccacagaagatggagtacgaaattacaaactactcagaaagacatacagaacttccaggtcatttcattggcctcaatacagtagataaactagaggagtccccgttaagggactttgttaagagtcacggtggtcacacggtcatatccaagatcctgatagcaaataatggtattgccgccgtgaaagaaattagatccgtcagaaaatgggcatacgagacgttcggcgatgacagaaccgtccaattcgtcgccatggccaccccagaagatctggaggccaacgcagaatatatccgtatggccgatcaatacattgaagtgccaggtggtactaataataacaactacgctaacgtagacttgatcgtagacatcgccgaaagagcagacgtagacgccgtatgggctggctggggtcacgcctccgagaatccactattgcctgaaaaattgtcccagtctaagaggaaagtcatctttattgggcctccaggtaacgccatgaggtctttaggtgataaaatctcctctaccattgtcgctcaaagtgctaaagtcccatgtattccatggtctggtaccggtgttgacaccgttcacgtggacgagaaaaccggtctggtctctgtcgacgatgacatctatcaaaagggttgttgtacctctcctgaagatggtttacaaaaggccaagcgtattggttttcctgtcatgattaaggcatccgaaggtggtggtggtaaaggtatcagacaagttgaacgtgaagaagatttcatcgctttataccaccaggcagccaacgaaattccaggctcccccattttcatcatgaagttggccggtagagcgcgtcacttggaagttcaactgctagcagatcagtacggtacaaatatttccttgttcggtagagactgttccgttcagagacgtcatcaaaaaattatcgaagaagcaccagttacaattgccaaggctgaaacatttcacgagatggaaaaggctgccgtcagactggggaaactagtcggttatgtctctgccggtaccgtggagtatctatattctcatgatgatggaaaattctactttttagaattgaacccaagattacaagtcgagcatccaacaacggaaatggtctccggtgttaacttacctgcagctcaattacaaatcgctatgggtatccctatgcatagaataagtgacattagaactttatatggtatgaatcctcattctgcctcagaaatcgatttcgaattcaaaactcaagatgccaccaagaaacaaagaagacctattccaaagggtcattgtaccgcttgtcgtatcacatcagaagatccaaacgatggattcaagccatcgggtggtactttgcatgaactaaacttccgttcttcctctaatgtttggggttacttctccgtgggtaacaatggtaatattcactccttttcggactctcagttcggccatatttttgcttttggtgaaaatagacaagcttccaggaaacacatggttgttgccctgaaggaattgtccattaggggtgatttcagaactactgtggaatacttgatcaaacttttggaaactgaagatttcgaggataacactattaccaccggttggttggacgatttgattactcataaaatgaccgctgaaaagcctgatccaactcttgccgtcatttgcggtgccgctacaaaggctttcttagcatctgaagaagcccgccacaagtatatcgaatccttacaaaagggacaagttctatctaaagacctactgcaaactatgttccctgtagattttatccatgagggtaaaagatacaagttcaccgtagctaaatccggtaatgaccgttacacattatttatcaatggttctaaatgtgatatcatactgcgtcaactatctgatggtggtcttttgattgccataggcggtaaatcgcataccatctattggaaagaagaagttgctgctacaagattatccgttgactctatgactactttgttggaagttgaaaacgatccaacccagttgcgtactccatcccctggtaaattggttaaattcttggtggaaaatggtgaacacattatcaagggccaaccatatgcagaaattgaagttatgaaaatgcaaatgcctttggtttctcaagaaaatggtatcgtccagttattaaagcaacctggttctaccattgttgcaggtgatatcatggctattatgactcttgacgatccatccaaggtcaagcacgctctaccatttgaaggtatgctgccagattttggttctccagttatcgaaggaaccaaacctgcctataaattcaagtcattagtgtctactttggaaaacattttgaagggttatgacaaccaagttattatgaacgcttccttgcaacaattgatagaggttttgagaaatccaaaactgccttactcagaatggaaactacacatctctgctttacattcaagattgcctgctaagctagatgaacaaatggaagagttagttgcacgttctttgagacgtggtgctgttttcccagctagacaattaagtaaattgattgatatggccgtgaagaatcctgaatacaaccccgacaaattgctgggcgccgtcgtggaaccattggcggatattgctcataagtactctaacgggttagaagcccatgaacattctatatttgtccatttcttggaagaatattacgaagttgaaaagttattcaatggtccaaatgttcgtgaggaaaatatcattctgaaattgcgtgatgaaaaccctaaagatctagataaagttgcgctaactgttttgtctcattcgaaagtttcagcgaagaataacctgatcctagctatcttgaaacattatcaaccattgtgcaagttatcttctaaagtttctgccattttctctactcctctacaacatattgttgaactagaatctaaggctaccgctaaggtcgctctacaagcaagagaaattttgattcaaggcgctttaccttcggtcaaggaaagaactgaacaaattgaacatatcttaaaatcctctgttgtgaaggttgcctatggctcatccaatccaaagcgctctgaaccagatttgaatatcttgaaggacttgatcgattctaattacgttgtgttcgatgttttacttcaattcctaacccatcaagacccagttgtgactgctgcagctgctcaagtctatattcgtcgtgcttatcgtgcttacaccataggagatattagagttcacgaaggtgtcacagttccaattgttgaatggaaattccaactaccttcagctgcgttctccacctttccaactgttaaatctaaaatgggtatgaacagggctgtttctgtttcagatttgtcatatgttgcaaacagtcagtcatctccgttaagagaaggtattttgatggctgtggatcatttagatgatgttgatgaaattttgtcacaaagtttggaagttattcctcgtcaccaatcttcttctaacggacctgctcctgatcgttctggtagctccgcatcgttgagtaatgttgctaatgtttgtgttgcttctacagaaggtttcgaatctgaagaggaaattttggtaaggttgagagaaattttggatttgaataagcaggaattaatcaatgcttctatccgtcgtatcacatttatgttcggttttaaagatgggtcttatccaaagtattatacttttaacggtccaaattataacgaaaatgaaacaattcgtcacattgagccggctttggccttccaactggaattaggaagattgtccaacttcaacattaaaccaattttcactgataatagaaacatccatgtctacgaagctgttagtaagacttctccattggataagagattctttacaagaggtattattagaacgggtcatatccgtgatgacatttctattcaagaatatctgacttctgaagctaacagattgatgagtgatatattggataatttagaagtcaccgacacttcaaattctgatttgaatcatatcttcatcaacttcattgcggtgtttgatatctctccagaagatgtcgaagccgccttcggtggtttcttagaaagatttggtaagagattgttgagattgcgtgtttcttctgccgaaattagaatcatcatcaaagatcctcaaacaggtgccccagtaccattgcgtgccttgatcaataacgtttctggttatgttatcaaaacagaaatgtacaccgaagtcaagaacgcaaaaggtgaatgggtatttaagtctttgggtaaacctggatccatgcatttaagacctattgctactccttaccctgttaaggaatggttgcaaccaaaacgttataaggcacacttgatgggtaccacatatgtctatgacttcccagaattattccgccaagcatcgtcatcccaatggaaaaatttctctgcagatgttaagttaacagatgatttctttatttccaacgagttgattgaagatgaaaacggcgaattaactgaggtggaaagagaacctggtgccaacgctattggtatggttgcctttaagattactgtaaagactcctgaatatccaagaggccgtcaatttgttgttgttgctaacgatatcacattcaagatcggttcctttggtccacaagaagacgaattcttcaataaggttactgaatatgctagaaagcgtggtatcccaagaatttacttggctgcaaactcaggtgccagaattggtatggctgaagagattgttccactatttcaagttgcatggaatgatgctgccaatccggacaagggcttccaatacttatacttaacaagtgaaggtatggaaactttaaagaaatttgacaaagaaaattctgttctcactgaacgtactgttataaacggtgaagaaagatttgtcatcaagacaattattggttctgaagatgggttaggtgtcgaatgtctacgtggatctggtttaattgctggtgcaacgtcaagggcttaccacgatatcttcactatcaccttagtcacttgtagatccgtcggtatcggtgcttatttggttcgtttgggtcaaagagctattcaggtcgaaggccagccaattattttaactggtgctcctgcaatcaacaaaatgctgggtagagaagtttatacttctaacttacaattgggtggtactcaaatcatgtataacaacggtgtttcacatttgactgctgttgacgatttagctggtgtagagaagattgttgaatggatgtcttatgttccagccaagcgtaatatgccagttcctatcttggaaactaaagacacatgggatagaccagttgatttcactccaactaatgatgaaacttacgatgtaagatggatgattgaaggtcgtgagactgaaagtggatttgaatatggtttgtttgataaagggtctttctttgaaactttgtcaggatgggccaaaggtgttgtcgttggtagagcccgtcttggtggtattccactgggtgttattggtgttgaaacaagaactgtcgagaacttgattcctgctgatccagctaatccaaatagtgctgaaacattaattcaagaacctggtcaagtttggcatccaaactccgccttcaagactgctcaagctatcaatgactttaacaacggtgaacaattgccaatgatgattttggccaactggagaggtttctctggtggtcaacgtgatatgttcaacgaagtcttgaagtatggttcgtttattgttgacgcattggtggattacaaacaaccaattattatctatatcccacctaccggtgaactaagaggtggttcatgggttgttgtcgatccaactatcaacgctgaccaaatggaaatgtatgccgacgtcaacgctagagctggtgttttggaaccacaaggtatggttggtatcaagttccgtagagaaaaattgctggacaccatgaacagattggatgacaagtacagagaattgagatctcaattatccaacaagagtttggctccagaagtacatcagcaaatatccaagcaattagctgatcgtgagagagaactattgccaatttacggacaaatcagtcttcaatttgctgatttgcacgataggtcttcacgtatggtggccaagggtgttatttctaaggaactggaatggaccgaggcacgtcgtttcttcttctggagattgagaagaagattgaacgaagaatatttgattaaaaggttgagccatcaggtaggcgaagcatcaagattagaaaagatcgcaagaattagatcgtggtaccctgcttcagtggaccatgaagatgataggcaagtcgcaacatggattgaagaaaactacaaaactttggacgataaactaaagggtttgaaattagagtcattcgctcaagacttagctaaaaagatcagaagcgaccatgacaatgctattgatggattatctgaagttatcaagatgttatctaccgatgataaagaaaaattgttgaagactttggtcaaataa

SEQ ID NO: 2 - protein, 2250 aa, Saccharomyces cerevisiae
MTIHLLYFHANRGQENMSEESLFESSPQKMEYEITNYSERHTELPGHFIGLNTVDKLEESPLRDFVKSHGGHTVISKILIANNGIAAVKEIRSVRKWAYETFGDDRTVQFVAMATPEDLEANAEYIRMADQYIEVPGGTNNNNYANVDLIVDIAERADVDAVWAGWGHASENPLLPEKLSQSKRKVIFIGPPGNAMRSLGDKISSTIVAQSAKVPCIPWSGTGVDTVHVDEKTGLVSVDDDIYQKGCCTSPEDGLQKAKRIGFPVMIKASEGGGGKGIRQVEREEDFIALYHQAANEIPGSPIFIMKLAGRARHLEVQLLADQYGTNISLFGRDCSVQRRHQKIIEEAPVTIAKAETFHEMEKAAVRLGKLVGYVSAGTVEYLYSHDDGKFYFLELNPRLQVEHPTTEMVSGVNLPAAQLQIAMGIPMHRISDIRTLYGMNPHSASEIDFEFKTQDATKKQRRPIPKGHCTACRITSEDPNDGFKPSGGTLHELNFRSSSNVWGYFSVGNNGNIHSFSDSQFGHIFAFGENRQASRKHMVVALKELSIRGDFRTTVEYLIKLLETEDFEDNTITTGWLDDLITHKMTAEKPDPTLAVICGAATKAFLASEEARHKYIESLQKGQVLSKDLLQTMFPVDFIHEGKRYKFTVAKSGNDRYTLFINGSKCDIILRQLSDGGLLIAIGGKSHTIYWKEEVAATRLSVDSMTTLLEVENDPTQLRTPSPGKLVKFLVENGEHIIKGQPYAEIEVMKMQMPLVSQENGIVQLLKQPGSTIVAGDIMAIMTLDDPSKVKHALPFEGMLPDFGSPVIEGTKPAYKFKSLVSTLENILKGYDNQVIMNASLQQLIEVLRNPKLPYSEWKLHISALHSRLPAKLDEQMEELVARSLRRGAVFPARQLSKLIDMAVKNPEYNPDKLLGAVVEPLADIAHKYSNGLEAHEHSIFVHFLEEYYEVEKLFNGPNVREENIILKLRDENPKDLDKVALTVLSHSKVSAKNNLILAILKHYQPLCKLSSKVSAIFSTPLQHIVELESKATAKVALQAREILIQGALPSVKERTEQIEHILKSSVVKVAYGSSNPKRSEPDLNILKDLIDSNYVVFDVLLQFLTHQDPVVTAAAAQVYIRRAYRAYTIGDIRVHEGVTVPIVEWKFQLPSAAFSTFPTVKSKMGMNRAVSVSDLSYVANSQSSPLREGILMAVDHLDDVDEILSQSLEVIPRHQSSSNGPAPDRSGSSASLSNVANVCVASTEGFESEEEILVRLREILDLNKQELINASIRRITFMFGFKDGSYPKYYTFNGPNYNENETIRHIEPALAFQLELGRLSNFNIKPIFTDNRNIHVYEAVSKTSPLDKRFFTRGIIRTGHIRDDISIQEYLTSEANRLMSDILDNLEVTDTSNSDLNHIFINFIAVFDISPEDVEAAFGGFLERFGKRLLRLRVSSAEIRIIIKDPQTGAPVPLRALINNVSGYVIKTEMYTEVKNAKGEWVFKSLGKPGSMHLRPIATPYPVKEWLQPKRYKAHLMGTTYVYDFPELFRQASSSQWKNFSADVKLTDDFFISNELIEDENGELTEVEREPGANAIGMVAFKITVKTPEYPRGRQFVVVANDITFKIGSFGPQEDEFFNKVTEYARKRGIPRIYLAANSGARIGMAEEIVPLFQVAWNDAANPDKGFQYLYLTSEGMETLKKFDKENSVLTERTVINGEERFVIKTIIGSEDGLGVECLRGSGLIAGATSRAYHDIFTITLVTCRSVGIGAYLVRLGQRAIQVEGQPIILTGAPAINKMLGREVYTSNLQLGGTQIMYNNGVSHLTAVDDLAGVEKIVEWMSYVPAKRNMPVPILETKDTWDRPVDFTPTNDETYDVRWMIEGRETESGFEYGLFDKGSFFETLSGWAKGVVVGRARLGGIPLGVIGVETRTVENLIPADPANPNSAETLIQEPGQVWHPNSAFKTAQAINDFNNGEQLPMMILANWRGFSGGQRDMFNEVLKYGSFIVDALVDYKQPIIIYIPPTGELRGGSWVVVDPTINADQMEMYADVNARAGVLEPQGMVGIKFRREKLLDTMNRLDDKYRELRSQLSNKSLAPEVHQQISKQLADRERELLPIYGQISLQFADLHDRSSRMVAKGVISKELEWTEARRFFFWRLRRRLNEEYLIKRLSHQVGEASRLEKIARIRSWYPASVDHEDDRQVATWIEENYKTLDDKLKGLKLESFAQDLAKKIRSDHDNAIDGLSEVIKMLSTDDKEKLLKTLVK

SEQ ID NO: 3 - DNA, 792 bp, Escherichia coli
  CDS (1)..(792)
atgggggaagcggtgatcgccgaagtatcgactcaactatcagaggtagttggcgtcatcgagcgccatctcgaaccgacgttgctggccgtacatttgtacggctccgcagtggatggcggcctgaagccacacagtgatattgatttgctggttacggtgaccgtaaggcttgatgaaacaacgcggcgagctttgatcaacgaccttttggaaacttcggcttcccctggagagagcgagattctccgcgctgtagaagtcaccattgttgtgcacgacgacatcattccgtggcgttatccagctaagcgcgaactgcaatttggagaatggcagcgcaatgacattcttgcaggtatcttcgagccagccacgatcgacattgatctggctatcttgctgacaaaagcaagagaacatagcgttgccttggtaggtccagcggcggaggaactctttgatccggttcctgaacaggatctatttgaggcgctaaatgaaaccttaacgctatggaactcgccgcccgactgggctggcgatgagcgaaatgtagtgcttacgttgtcccgcatttggtacagcgcagtaaccggcaaaatcgcgccgaaggatgtcgctgccgactgggcaatggagcgcctgccggcccagtatcagcccgtcatacttgaagctagacaggcttatcttggacaagaagaagatcgcttggcctcgcgcgcagatcagttggaagaatttgtccactacgtgaaaggcgagatcaccaaggtagtcggcaaataa

SEQ ID NO: 4 - protein, 263 aa, Escherichia coli
MGEAVIAEVSTQLSEVVGVIERHLEPTLLAVHLYGSAVDGGLKPHSDIDLLVTVTVRLDETTRRALINDLLETSASPGESEILRAVEVTIVVHDDIIPWRYPAKRELQFGEWQRNDILAGIFEPATIDIDLAILLTKAREHSVALVGPAAEELFDPVPEQDLFEALNETLTLWNSPPDWAGDERNVVLTLSRIWYSAVTGKIAPKDVAADWAMERLPAQYQPVILEARQAYLGQEEDRLASRADQLEEFVHYVKGEITKVVGK

SEQ ID NO: 5 - DNA, 14853 bp, Artificial Sequence
  full-sequence of pACC
  gene (4071)..(10823): ScACC1 (complement)
  gene (10776)..(10823): accD (complement)
  gene (11378)..(12169): aadA
  gene (12218)..(12940): TagRFP
tcacgacgttgtaaaacgacggccagtgaattcgagctcggtacccggggatcctctagagtcgacctgcaggcatgcaagcttggcgtaatcatggtcatagctgtttcctgtgtgaaattgttatccgctcacaattccacacaacatacgagccggaagcataaagtgtaaagcctggggtgcctaatgagtgagctaactcacattaattgcgttgcgctcactgcccgctttccagtcgggaaacctgtcgtgccagctgcattaatgaatcggccaacgcgcggggagaggcggtttgcgtattgggcgctcttccgcttcctcgctcactgactcgctgcgctcggtcgttcggctgcggcgagcggtatcagctcactcaaaggcggtaatacggttatccacagaatcaggggataacgcaggaaagaacatgtgagcaaaaggccagcaaaaggccaggaaccgtaaaaaggccgcgttgctggcgtttttccataggctccgcccccctgacgagcatcacaaaaatcgacgctcaagtcagaggtggcgaaacccgacaggactataaagataccaggcgtttccccctggaagctccctcgtgcgctctcctgttccgaccctgccgcttaccggatacctgtccgcctttctcccttcgggaagcgtggcgctttctcatagctcacgctgtaggtatctcagttcggtgtaggtcgttcgctccaagctgggctgtgtgcacgaaccccccgttcagcccgaccgctgcgccttatccggtaactatcgtcttgagtccaacccggtaagacacgacttatcgccactggcagcagccactggtaacaggattagcagagcgaggtatgtaggcggtgctacagagttcttgaagtggtggcctaactacggctacactagaagaacagtatttggtatctgcgctctgctgaagccagttaccttcggaaaaagagttggtagctcttgatccggcaaacaaaccaccgctggtagcggtggtttttttgtttgcaagcagcagattacgcgcagaaaaaaaggatctcaagaagatcctttgatcttttctacggggtctgacgctcagtggaacgaaaactcacgttaagggattttggtcatgagattatcaaaaaggatcttcacctagatccttttaaattaaaaatgaagttttaaatcaatctaaagtatatatgagtaaacttggtctgacagttaccaatgcttaatcagtgaggcacctatctcagcgatctgtctatttcgttcatccatagttgcctgactccccgtcgtgtagataactacgatacgggagggcttaccatctggccccagtgctgcaatgataccgcgagacccacgctcaccggctccagatttatcagcaataaaccagccagccggaagggccgagcgcagaagtggtcctgcaactttatccgcctccatccagtctattaattgttgccgggaagctagagtaagtagttcgccagttaatagtttgcgcaacgttgttgccattgctacaggcatcgtggtgtcacgctcgtcgtttggtatggcttcattcagctccggttcccaacgatcaaggcgagttacatgatcccccatgttgtgcaaaaaagcggttagctccttcggtcctccgatcgttgtcagaagtaagttggccgcagtgttatcactcatggttatggcagcactgcataattctcttactgtcatgccatccgtaagatgcttttctgtgactggtgagtactcaaccaagtcattctgagaatagtgtatgcggcgaccgagttgctcttgcccggcgtcaatacgggataataccgcgccacatagcagaactttaaaagtgctcatcattggaaaacgttcttcggggcgaaaactctcaaggatcttaccgctgttgagatccagttcgatgtaacccactcgtgcacccaactgatcttcagcatcttttactttcaccagcgtttctgggtgagcaaaaacaggaaggcaaaatgccgcaaaaaagggaataagggcgacacggaaatgttgaatactcatactcttcctttttcaatattattgaagcatttatcagggttattgtctcatgagcggatacatatttgaatgtatttagaaaaataaacaaataggggttccgcgcacatttccccgaaaagtgccacctgacgtctaagaaaccattattatcatgacattaacctataaaaataggcgtatcacgaggccctttcgtctgaagcaggaatcgctagtaatcgccggtcagccatacggcggtgaatccgttcccgggccttgtacacaccgcccgtcacactataggagctggccatgtttgaagtcattacccttaaccgtaaggagggggatgcctaaggctaggcttgcgactggagtgaagtcgtaacaaggtagccgtactggaaggtgcggctggatcacctccttttcagggagagctaatgcttatgcttattgggtattttggtttgacactgcttcacgcccaaaaagaaggcagctacgtctgagctaaacttggatatggaagtcttctttcgtttagggtgaagtaagaccaagctcatgagcttattatcctaggtcggaacaaattagttgatagtgataggatcccctttttgacgtccccatgcccccccccgtgtggtgtggcggcatggggatgtcaaaaggaaagggatggagtttttctcgcttttggcgtagcaggcctcccaaagggaggcccgcgcgacgggctattagctcagtggtagagcgcgcccctgataattgcgtcgttgtgcctgggctgtgagggctctcagccacatggatagttcaatgtgctcatcagcgcctgacccgaagatgtggatcatccaaggcacattagcatggcgtactcctcctgtttgaatcggagtttgaaaccaaacaaacttctcctcaggaggatagatggggcgattcaggtgagatcccatgtagatctaactttctattcactcgtgggatccgggcggtccggggggggcactacggctcctctcttctcgagaatccatacatcccttatcagtgtatggagagctatctctcgagcacaggttgaggttcgtcctcaatgggaaaatggagcacctaacaacgcatcttcacagaccaagaactacgagatcaccctttcattctggggtgacggagggatcgtaccattcgagcctttttttcatgcttttcccggcggtctggagaaagcagcaatcaataggacttccctaatcctcccttcctgaaaggaagaacgtgaaattctttttcctttccgcagggaccaggaggttggatctagccataagaggaatgcttggtataaataagccacttcttggtcttcgactccctaagtcactacgagcgccctcgatcagtgcaatgggatgtggctatttatctatctcttgactcgaaatgggagcagagcaggtttgaaaaaggatcttagagtgtctagggttgggccaggagggtctcttaacgccttcctttttctgcccatcggagttatttcccaaggacttgccatggtaagggggagaaggggaagaagcacacttgaagagcgcagtacaacggagagttgtatgctgcgttcgggaaggatgaatcgctcccgaaaaggagtctattgattctctcccaattggttggatcgtaggggcgatgatttacttcacgggcgaggtctctggttcaagtccaggatggcccagctgcgccagggaaaagaatagaagaagcatctgacgtttcctcagcgtcgacaattcaatggaagcaatgataaaaaaatacaaatagaaaaggaaagggaggaaatacaaaaaaatagaagagaaaagtcatacaaagttatatacaaatgactacccccctttttgtatttccttaatttatttccttaattgaatttcggatccttatttgaccaaagtcttcaacaatttttctttatcatcggtagataacatcttgataacttcagataatccatcaatagcattgtcatggtcgcttctgatctttttagctaagtcttgagcgaatgactctaatttcaaaccctttagtttatcgtccaaagttttgtagttttcttcaatccatgttgcgacttgcctatcatcttcatggtccactgaagcagggtaccacgatctaattcttgcgatcttttctaatcttgatgcttcgcctacctgatggctcaaccttttaatcaaatattcttcgttcaatcttcttctcaatctccagaagaagaaacgacgtgcctcggtccattccagttccttagaaataacacccttggccaccatacgtgaagacctatcgtgcaaatcagcaaattgaagactgatttgtccgtaaattggcaatagttctctctcacgatcagctaattgcttggatatttgctgatgtacttctggagccaaactcttgttggataattgagatctcaattctctgtacttgtcatccaatctgttcatggtgtccagcaatttttctctacggaacttgataccaaccataccttgtggttccaaaacaccagctctagcgttgacgtcggcatacatttccatttggtcagcgttgatagttggatcgacaacaacccatgaaccacctcttagttcaccggtaggtgggatatagataataattggttgtttgtaatccaccaatgcgtcaacaataaacgaaccatacttcaagacttcgttgaacatatcacgttgaccaccagagaaacctctccagttggccaaaatcatcattggcaattgttcaccgttgttaaagtcattgatagcttgagcagtcttgaaggcggagtttggatgccaaacttgaccaggttcttgaattaatgtttcagcactatttggattagctggatcagcaggaatcaagttctcgacagttcttgtttcaacaccaataacacccagtggaataccaccaagacgggctctaccaacgacaacacctttggcccatcctgacaaagtttcaaagaaagaccctttatcaaacaaaccatattcaaatccactttcagtctcacgaccttcaatcatccatcttacatcgtaagtttcatcattagttggagtgaaatcaactggtctatcccatgtgtctttagtttccaagataggaactggcatattacgcttggctggaacataagacatccattcaacaatcttctctacaccagctaaatcgtcaacagcagtcaaatgtgaaacaccgttgttatacatgatttgagtaccacccaattgtaagttagaagtataaacttctctacccagcattttgttgattgcaggagcaccagttaaaataattggctggccttcgacctgaatagctctttgacccaaacgaaccaaataagcaccgataccgacggatctacaagtgactaaggtgatagtgaagatatcgtggtaagcccttgacgttgcaccagcaattaaaccagatccacgtagacattcgacacctaacccatcttcagaaccaataattgtcttgatgacaaatctttcttcaccgtttataacagtacgttcagtgagaacagaattttctttgtcaaatttctttaaagtttccataccttcacttgttaagtataagtattggaagcccttgtccggattggcagcatcattccatgcaacttgaaatagtggaacaatctcttcagccataccaattctggcacctgagtttgcagccaagtaaattcttgggataccacgctttctagcatattcagtaaccttattgaagaattcgtcttcttgtggaccaaaggaaccgatcttgaatgtgatatcgttagcaacaacaacaaattgacggcctcttggatattcaggagtctttacagtaatcttaaaggcaaccataccaatagcgttggcaccaggttctctttccacctcagttaattcgccgttttcatcttcaatcaactcgttggaaataaagaaatcatctgttaacttaacatctgcagagaaatttttccattgggatgacgatgcttggcggaataattctgggaagtcatagacatatgtggtacccatcaagtgtgccttataacgttttggttgcaaccattccttaacagggtaaggagtagcaataggtcttaaatgcatggatccaggtttacccaaagacttaaatacccattcaccttttgcgttcttgacttcggtgtacatttctgttttgataacataaccagaaacgttattgatcaaggcacgcaatggtactggggcacctgtttgaggatctttgatgatgattctaatttcggcagaagaaacacgcaatctcaacaatctcttaccaaatctttctaagaaaccaccgaaggcggcttcgacatcttctggagagatatcaaacaccgcaatgaagttgatgaagatatgattcaaatcagaatttgaagtgtcggtgacttctaaattatccaatatatcactcatcaatctgttagcttcagaagtcagatattcttgaatagaaatgtcatcacggatatgacccgttctaataatacctcttgtaaagaatctcttatccaatggagaagtcttactaacagcttcgtagacatggatgtttctattatcagtgaaaattggtttaatgttgaagttggacaatcttcctaattccagttggaaggccaaagccggctcaatgtgacgaattgtttcattttcgttataatttggaccgttaaaagtataatactttggataagacccatctttaaaaccgaacataaatgtgatacgacggatagaagcattgattaattcctgcttattcaaatccaaaatttctctcaaccttaccaaaatttcctcttcagattcgaaaccttctgtagaagcaacacaaacattagcaacattactcaacgatgcggagctaccagaacgatcaggagcaggtccgttagaagaagattggtgacgaggaataacttccaaactttgtgacaaaatttcatcaacatcatctaaatgatccacagccatcaaaataccttctcttaacggagatgactgactgtttgcaacatatgacaaatctgaaacagaaacagccctgttcatacccattttagatttaacagttggaaaggtggagaacgcagctgaaggtagttggaatttccattcaacaattggaactgtgacaccttcgtgaactctaatatctcctatggtgtaagcacgataagcacgacgaatatagacttgagcagctgcagcagtcacaactgggtcttgatgggttaggaattgaagtaaaacatcgaacacaacgtaattagaatcgatcaagtccttcaagatattcaaatctggttcagagcgctttggattggatgagccataggcaaccttcacaacagaggattttaagatatgttcaatttgttcagttctttccttgaccgaaggtaaagcgccttgaatcaaaatttctcttgcttgtagagcgaccttagcggtagccttagattctagttcaacaatatgttgtagaggagtagagaaaatggcagaaactttagaagataacttgcacaatggttgataatgtttcaagatagctaggatcaggttattcttcgctgaaactttcgaatgagacaaaacagttagcgcaactttatctagatctttagggttttcatcacgcaatttcagaatgatattttcctcacgaacatttggaccattgaataacttttcaacttcgtaatattcttccaagaaatggacaaatatagaatgttcatgggcttctaacccgttagagtacttatgagcaatatccgccaatggttccacgacggcgcccagcaatttgtcggggttgtattcaggattcttcacggccatatcaatcaatttacttaattgtctagctgggaaaacagcaccacgtctcaaagaacgtgcaactaactcttccatttgttcatctagcttagcaggcaatcttgaatgtaaagcagagatgtgtagtttccattctgagtaaggcagttttggatttctcaaaacctctatcaattgttgcaaggaagcgttcataataacttggttgtcataacccttcaaaatgttttccaaagtagacactaatgacttgaatttataggcaggtttggttccttcgataactggagaaccaaaatctggcagcataccttcaaatggtagagcgtgcttgaccttggatggatcgtcaagagtcataatagccatgatatcacctgcaacaatggtagaaccaggttgctttaataactggacgataccattttcttgagaaaccaaaggcatttgcattttcataacttcaatttctgcatatggttggcccttgataatgtgttcaccattttccaccaagaatttaaccaatttaccaggggatggagtacgcaactgggttggatcgttttcaacttccaacaaagtagtcatagagtcaacggataatcttgtagcagcaacttcttctttccaatagatggtatgcgatttaccgcctatggcaatcaaaagaccaccatcagatagttgacgcagtatgatatcacatttagaaccattgataaataatgtgtaacggtcattaccggatttagctacggtgaacttgtatcttttaccctcatggataaaatctacagggaacatagtttgcagtaggtctttagatagaacttgtcccttttgtaaggattcgatatacttgtggcgggcttcttcagatgctaagaaagcctttgtagcggcaccgcaaatgacggcaagagttggatcaggcttttcagcggtcattttatgagtaatcaaatcgtccaaccaaccggtggtaatagtgttatcctcgaaatcttcagtttccaaaagtttgatcaagtattccacagtagttctgaaatcacccctaatggacaattccttcagggcaacaaccatgtgtttcctggaagcttgtctattttcaccaaaagcaaaaatatggccgaactgagagtccgaaaaggagtgaatattaccattgttacccacggagaagtaaccccaaacattagaggaagaacggaagtttagttcatgcaaagtaccacccgatggcttgaatccatcgtttggatcttctgatgtgatacgacaagcggtacaatgaccctttggaataggtcttctttgtttcttggtggcatcttgagttttgaattcgaaatcgatttctgaggcagaatgaggattcataccatataaagttctaatgtcacttattctatgcatagggatacccatagcgatttgtaattgagctgcaggtaagttaacaccggagaccatttccgttgttggatgctcgacttgtaatcttgggttcaattctaaaaagtagaattttccatcatcatgagaatatagatactccacggtaccggcagagacataaccgactagtttccccagtctgacggcagccttttccatctcgtgaaatgtttcagccttggcaattgtaactggtgcttcttcgataattttttgatgacgtctctgaacggaacagtctctaccgaacaaggaaatatttgtaccgtactgatctgctagcagttgaacttccaagtgacgcgctctaccggccaacttcatgatgaaaatgggggagcctggaatttcgttggctgcctggtggtataaagcgatgaaatcttcttcacgttcaacttgtctgatacctttaccaccaccaccttcggatgccttaatcatgacaggaaaaccaatacgcttggccttttgtaaaccatcttcaggagaggtacaacaacccttttgatagatgtcatcgtcgacagagaccagaccggttttctcgtccacgtgaacggtgtcaacaccggtaccagaccatggaatacatgggactttagcactttgagcgacaatggtagaggagattttatcacctaaagacctcatggcgttacctggaggcccaataaagatgactttcctcttagactgggacaatttttcaggcaatagtggattctcggaggcgtgaccccagccagcccatacggcgtctacgtctgctctttcggcgatgtctacgatcaagtctacgttagcgtagttgttattattagtaccacctggcacttcaatgtattgatcggccatacggatatattctgcgttggcctccagatcttctggggtggccatggcgacgaattggacggttctgtcatcgccgaacgtctcgtatgcccattttctgacggatctaatttctttcacggcggcaataccattatttgctatcaggatcttggatatgaccgtgtgaccaccgtgactcttaacaaagtcccttaacggggactcctctagtttatctactgtattgaggccaatgaaatgacctggaagttctgtatgtctttctgagtagtttgtaatttcgtactccatcttctgtggagaagactcgaataagctttcttcgctcatgttttcttgccccctatttgcatgaaaatacaatagatgaatagtcattcgctataaaattatttatttgaatatcttatttcctatcagactaagcatagaaatccaatcactaggattattaactaataagtattgtgagtattgaaaaaaagttctgaatctgggggaacacttcactatatattaatatgttggaaccccctttatattatttaaaataatataataatataatttttaataaagggcggcttctcctatgtcggagctcgtttaaacgagctcgctcccccgccgtcgttcaatgtgaatggataagaggctcgtgggattgacgtgagggggcagggatggctatatttctgggagaattaaccgatcgacgtgcaagcggacatttattttaaattcgataatttttgcaaaaacatttcgacatatttatttattttattattatgacatgtttttttggggtacagtctatgcctcgggcatccaagcagcaagcgcgttacgccgtgggtcgatgtttgatgttatggagcagcaacgatgttacgcagcagggcagtcgccctaaaacaaagttaaacatcatgggggaagcggtgatcgccgaagtatcgactcaactatcagaggtagttggcgtcatcgagcgccatctcgaaccgacgttgctggccgtacatttgtacggctccgcagtggatggcggcctgaagccacacagtgatattgatttgctggttacggtgaccgtaaggcttgatgaaacaacgcggcgagctttgatcaacgaccttttggaaacttcggcttcccctggagagagcgagattctccgcgctgtagaagtcaccattgttgtgcacgacgacatcattccgtggcgttatccagctaagcgcgaactgcaatttggagaatggcagcgcaatgacattcttgcaggtatcttcgagccagccacgatcgacattgatctggctatcttgctgacaaaagcaagagaacatagcgttgccttggtaggtccagcggcggaggaactctttgatccggttcctgaacaggatctatttgaggcgctaaatgaaaccttaacgctatggaactcgccgcccgactgggctggcgatgagcgaaatgtagtgcttacgttgtcccgcatttggtacagcgcagtaaccggcaaaatcgcgccgaaggatgtcgctgccgactgggcaatggagcgcctgccggcccagtatcagcccgtcatacttgaagctagacaggcttatcttggacaagaagaagatcgcttggcctcgcgcgcagatcagttggaagaatttgtccactacgtgaaaggcgagatcaccaaggtagtcggcaaataaacccaaataatgttttaaaattttaaaaataatgtaggaggaaaaattatggtgagtaaaggtgaagagttgattaaagagaacatgcatatgaagttatacatggagggaactgtcaataatcaccactttaagtgtacatcagagggtgagggaaagccatacgagggaacccaaactatgagaatcaaagtagtggagggaggtcctcttccatttgcttttgatatactagcaacaagtttcatgtatggttccaggaccttcattaaccatactcagggaatccctgacttctttaaacagtcttttcctgaaggttttacatgggagagggttaccacttacgaggacggtggagtcttgacagcaacccaggacacttcattacaagatggatgcctaatatacaatgtgaaaattaggggtgtgaatttccctagtaacggaccagttatgcagaagaaaacactaggttgggaagctaatactgaaatgttgtaccctgccgacggaggtttagaaggtagatccgacatggcccttaagctagtcggaggtggacacttgatctgtaactttaaaaccacatataggtctaagaagccagcaaagaatctaaaaatgcctggtgtttactatgtggaccatagactagaaaggataaaagaagcagacaaagaaacttacgtggagcaacatgaggtcgccgtcgctaggtattgcgacttaccttccaagctaggtcacaaattgaactccggactctagggatccaaacagtagacattagcagataaattagcaggaaataaagaaggataaggagaaagaactcaagtaattatccttcgttctcttaattgaattgcaattaaactcggcccaatcttttactaaaaggattgagccgaatacaacaaagattctattgcatatattttgactaagtatatacttacctagatatacaagatttgaaatacaaaatctagagcatgcgcgatcgcgctgattgacgcgccctcggggggatatagctcagttggtagagctccgctcttgcaattgggtcgttgcgattacgggttggctgtctaattgtccaggcggtaatggtagtatcttgtacctgaaccggtggctcactttttctaagtaatggggaagaggactgaaacatgccactgaaagactctactgagacaaaaagatgggctgtcaaaaaggtagaggaggtaggatgggcagttggtcagatctagtatggatcgtacatggacgatagttggagtcggcggctctcctaggcttccctcatctgggatccctggggaagaggatcaagtgtggcccttgcgaatagcttgatgcactatctcccttcaaccctttgagcgaaatgtggcaaaaggaaggaaaatccatggaccgaccccattatctccaccccgtaggaactacgagatcaccccaaggacgccttcggcgtccaggggtcacggaccgaccatagaccctgttcaataagtggaacacattagccgtccgctctccggttgggcagtaagggtcggagaagggcaatcactcgttcttaaaaccagcattcttaagtttaagatcaaagagtcgggcggaaaaaggggagagctccccgttcctggttctcctgtagctggattccccggaaccacaagaatccttagaatgggattccaactcagcaccttttgttttgagattttgagaagagttgctctttggagagcacagtacgatgaaagttgtaagctgtgttcgggggggagttattgtctatcgttggcctctatggtagaacccgtcggggaggcctgagaggcggtggtttaccctgtggcggatgtcagcggttcgagtccgcttatctccagcccgtgaacttagcggatactatgatagcaccgaattttgccaattcggcagttcgatctatgatttcgcattcatggacgttgataagatccttccatttagtagcaccttaggatggcatagccttaacgttaatggcgaggttcaaaagaggaaaggcttgcggtggatacctaggtacccagagacgaggaagggcgtagcaagcgacgaaatgcttcggggagttgaaaataagcatagatccggagattcccaaataggtcaaccttttgaactgcctgctgaatccatgagcaggcaagagacaacctggcgaactgaaacatcttagtagccagaggaaaagaaagcaaaagcgattcccgtagtagcggcgagcgaaatgggagcagcctaaaccgtgaaaacggggttgtgggagagcaatacaagcgttgtgctgctaggcgaagcggttgagtgccgcaccctagatggctaaagtccagtagccgaaagcatcactagcttacgctctgacccgagtagcatggggcacgtggaatcccgtgtgaatcagcaaggaccaccttgcaaggctaaatactcctgggtgaccgatagcgaagtagtaccgtgagggaaaggtgaaaagaacccccagtgggtagtgaaatagaacgtgaaaccgtgctgagctcccaagcagtgggaggggaaagtgatctctgaccgcgtgcctgttgaagaatgagccggcgactcataggcagtggcttggttaa

SEQ ID NO: 6 - DNA, 20844 bp, Artificial Sequence
  full-sequence of pACC-GD
  gene (4071)..(10823): ScACC1 (complement)
  gene (10776)..(10823): accD (complement)
  gene (11378)..(12169): aadA
  gene (12218)..(12940): TagRFP
  gene (14553)..(18659): OsCas9
tcacgacgttgtaaaacgacggccagtgaattcgagctcggtacccggggatcctctagagtcgacctgcaggcatgcaagcttggcgtaatcatggtcatagctgtttcctgtgtgaaattgttatccgctcacaattccacacaacatacgagccggaagcataaagtgtaaagcctggggtgcctaatgagtgagctaactcacattaattgcgttgcgctcactgcccgctttccagtcgggaaacctgtcgtgccagctgcattaatgaatcggccaacgcgcggggagaggcggtttgcgtattgggcgctcttccgcttcctcgctcactgactcgctgcgctcggtcgttcggctgcggcgagcggtatcagctcactcaaaggcggtaatacggttatccacagaatcaggggataacgcaggaaagaacatgtgagcaaaaggccagcaaaaggccaggaaccgtaaaaaggccgcgttgctggcgtttttccataggctccgcccccctgacgagcatcacaaaaatcgacgctcaagtcagaggtggcgaaacccgacaggactataaagataccaggcgtttccccctggaagctccctcgtgcgctctcctgttccgaccctgccgcttaccggatacctgtccgcctttctcccttcgggaagcgtggcgctttctcatagctcacgctgtaggtatctcagttcggtgtaggtcgttcgctccaagctgggctgtgtgcacgaaccccccgttcagcccgaccgctgcgccttatccggtaactatcgtcttgagtccaacccggtaagacacgacttatcgccactggcagcagccactggtaacaggattagcagagcgaggtatgtaggcggtgctacagagttcttgaagtggtggcctaactacggctacactagaagaacagtatttggtatctgcgctctgctgaagccagttaccttcggaaaaagagttggtagctcttgatccggcaaacaaaccaccgctggtagcggtggtttttttgtttgcaagcagcagattacgcgcagaaaaaaaggatctcaagaagatcctttgatcttttctacggggtctgacgctcagtggaacgaaaactcacgttaagggattttggtcatgagattatcaaaaaggatcttcacctagatccttttaaattaaaaatgaagttttaaatcaatctaaagtatatatgagtaaacttggtctgacagttaccaatgcttaatcagtgaggcacctatctcagcgatctgtctatttcgttcatccatagttgcctgactccccgtcgtgtagataactacgatacgggagggcttaccatctggccccagtgctgcaatgataccgcgagacccacgctcaccggctccagatttatcagcaataaaccagccagccggaagggccgagcgcagaagtggtcctgcaactttatccgcctccatccagtctattaattgttgccgggaagctagagtaagtagttcgccagttaatagtttgcgcaacgttgttgccattgctacaggcatcgtggtgtcacgctcgtcgtttggtatggcttcattcagctccggttcccaacgatcaaggcgagttacatgatcccccatgttgtgcaaaaaagcggttagctccttcggtcctccgatcgttgtcagaagtaagttggccgcagtgttatcactcatggttatggcagcactgcataattctcttactgtcatgccatccgtaagatgcttttctgtgactggtgagtactcaaccaagtcattctgagaatagtgtatgcggcgaccgagttgctcttgcccggcgtcaatacgggataataccgcgccacatagcagaactttaaaagtgctcatcattggaaaacgttcttcggggcgaaaactctcaaggatcttaccgctgttgagatccagttcgatgtaacccactcgtgcacccaactgatcttcagcatcttttactttcaccagcgtttctgggtgagcaaaaacaggaaggcaaaatgccgcaaaaaagggaataagggcgacacggaaatgttgaatactcatactcttcctttttcaatattattgaagcatttatcagggttattgtctcatgagcggatacatatttgaatgtatttagaaaaataaacaaataggggttccgcgcacatttccccgaaaagtgccacctgacgtctaagaaaccattattatcatgacattaacctataaaaataggcgtatcacgaggccctttcgtctgaagcaggaatcgctagtaatcgccggtcagccatacggcggtgaatccgttcccgggccttgtacacaccgcccgtcacactataggagctggccatgtttgaagtcattacccttaaccgtaaggagggggatgcctaaggctaggcttgcgactggagtgaagtcgtaacaaggtagccgtactggaaggtgcggctggatcacctccttttcagggagagctaatgcttatgcttattgggtattttggtttgacactgcttcacgcccaaaaagaaggcagctacgtctgagctaaacttggatatggaagtcttctttcgtttagggtgaagtaagaccaagctcatgagcttattatcctaggtcggaacaaattagttgatagtgataggatcccctttttgacgtccccatgcccccccccgtgtggtgtggcggcatggggatgtcaaaaggaaagggatggagtttttctcgcttttggcgtagcaggcctcccaaagggaggcccgcgcgacgggctattagctcagtggtagagcgcgcccctgataattgcgtcgttgtgcctgggctgtgagggctctcagccacatggatagttcaatgtgctcatcagcgcctgacccgaagatgtggatcatccaaggcacattagcatggcgtactcctcctgtttgaatcggagtttgaaaccaaacaaacttctcctcaggaggatagatggggcgattcaggtgagatcccatgtagatctaactttctattcactcgtgggatccgggcggtccggggggggcactacggctcctctcttctcgagaatccatacatcccttatcagtgtatggagagctatctctcgagcacaggttgaggttcgtcctcaatgggaaaatggagcacctaacaacgcatcttcacagaccaagaactacgagatcaccctttcattctggggtgacggagggatcgtaccattcgagcctttttttcatgcttttcccggcggtctggagaaagcagcaatcaataggacttccctaatcctcccttcctgaaaggaagaacgtgaaattctttttcctttccgcagggaccaggaggttggatctagccataagaggaatgcttggtataaataagccacttcttggtcttcgactccctaagtcactacgagcgccctcgatcagtgcaatgggatgtggctatttatctatctcttgactcgaaatgggagcagagcaggtttgaaaaaggatcttagagtgtctagggttgggccaggagggtctcttaacgccttcctttttctgcccatcggagttatttcccaaggacttgccatggtaagggggagaaggggaagaagcacacttgaagagcgcagtacaacggagagttgtatgctgcgttcgggaaggatgaatcgctcccgaaaaggagtctattgattctctcccaattggttggatcgtaggggcgatgatttacttcacgggcgaggtctctggttcaagtccaggatggcccagctgcgccagggaaaagaatagaagaagcatctgacgtttcctcagcgtcgacaattcaatggaagcaatgataaaaaaatacaaatagaaaaggaaagggaggaaatacaaaaaaatagaagagaaaagtcatacaaagttatatacaaatgactacccccctttttgtatttccttaatttatttccttaattgaatttcggatccttatttgaccaaagtcttcaacaatttttctttatcatcggtagataacatcttgataacttcagataatccatcaatagcattgtcatggtcgcttctgatctttttagctaagtcttgagcgaatgactctaatttcaaaccctttagtttatcgtccaaagttttgtagttttcttcaatccatgttgcgacttgcctatcatcttcatggtccactgaagcagggtaccacgatctaattcttgcgatcttttctaatcttgatgcttcgcctacctgatggctcaaccttttaatcaaatattcttcgttcaatcttcttctcaatctccagaagaagaaacgacgtgcctcggtccattccagttccttagaaataacacccttggccaccatacgtgaagacctatcgtgcaaatcagcaaattgaagactgatttgtccgtaaattggcaatagttctctctcacgatcagctaattgcttggatatttgctgatgtacttctggagccaaactcttgttggataattgagatctcaattctctgtacttgtcatccaatctgttcatggtgtccagcaatttttctctacggaacttgataccaaccataccttgtggttccaaaacaccagctctagcgttgacgtcggcatacatttccatttggtcagcgttgatagttggatcgacaacaacccatgaaccacctcttagttcaccggtaggtgggatatagataataattggttgtttgtaatccaccaatgcgtcaacaataaacgaaccatacttcaagacttcgttgaacatatcacgttgaccaccagagaaacctctccagttggccaaaatcatcattggcaattgttcaccgttgttaaagtcattgatagcttgagcagtcttgaaggcggagtttggatgccaaacttgaccaggttcttgaattaatgtttcagcactatttggattagctggatcagcaggaatcaagttctcgacagttcttgtttcaacaccaataacacccagtggaataccaccaagacgggctctaccaacgacaacacctttggcccatcctgacaaagtttcaaagaaagaccctttatcaaacaaaccatattcaaatccactttcagtctcacgaccttcaatcatccatcttacatcgtaagtttcatcattagttggagtgaaatcaactggtctatcccatgtgtctttagtttccaagataggaactggcatattacgcttggctggaacataagacatccattcaacaatcttctctacaccagctaaatcgtcaacagcagtcaaatgtgaaacaccgttgttatacatgatttgagtaccacccaattgtaagttagaagtataaacttctctacccagcattttgttgattgcaggagcaccagttaaaataattggctggccttcgacctgaatagctctttgacccaaacgaaccaaataagcaccgataccgacggatctacaagtgactaaggtgatagtgaagatatcgtggtaagcccttgacgttgcaccagcaattaaaccagatccacgtagacattcgacacctaacccatcttcagaaccaataattgtcttgatgacaaatctttcttcaccgtttataacagtacgttcagtgagaacagaattttctttgtcaaatttctttaaagtttccataccttcacttgttaagtataagtattggaagcccttgtccggattggcagcatcattccatgcaacttgaaatagtggaacaatctcttcagccataccaattctggcacctgagtttgcagccaagtaaattcttgggataccacgctttctagcatattcagtaaccttattgaagaattcgtcttcttgtggaccaaaggaaccgatcttgaatgtgatatcgttagcaacaacaacaaattgacggcctcttggatattcaggagtctttacagtaatcttaaaggcaaccataccaatagcgttggcaccaggttctctttccacctcagttaattcgccgttttcatcttcaatcaactcgttggaaataaagaaatcatctgttaacttaacatctgcagagaaatttttccattgggatgacgatgcttggcggaataattctgggaagtcatagacatatgtggtacccatcaagtgtgccttataacgttttggttgcaaccattccttaacagggtaaggagtagcaataggtcttaaatgcatggatccaggtttacccaaagacttaaatacccattcaccttttgcgttcttgacttcggtgtacatttctgttttgataacataaccagaaacgttattgatcaaggcacgcaatggtactggggcacctgtttgaggatctttgatgatgattctaatttcggcagaagaaacacgcaatctcaacaatctcttaccaaatctttctaagaaaccaccgaaggcggcttcgacatcttctggagagatatcaaacaccgcaatgaagttgatgaagatatgattcaaatcagaatttgaagtgtcggtgacttctaaattatccaatatatcactcatcaatctgttagcttcagaagtcagatattcttgaatagaaatgtcatcacggatatgacccgttctaataatacctcttgtaaagaatctcttatccaatggagaagtcttactaacagcttcgtagacatggatgtttctattatcagtgaaaattggtttaatgttgaagttggacaatcttcctaattccagttggaaggccaaagccggctcaatgtgacgaattgtttcattttcgttataatttggaccgttaaaagtataatactttggataagacccatctttaaaaccgaacataaatgtgatacgacggatagaagcattgattaattcctgcttattcaaatccaaaatttctctcaaccttaccaaaatttcctcttcagattcgaaaccttctgtagaagcaacacaaacattagcaacattactcaacgatgcggagctaccagaacgatcaggagcaggtccgttagaagaagattggtgacgaggaataacttccaaactttgtgacaaaatttcatcaacatcatctaaatgatccacagccatcaaaataccttctcttaacggagatgactgactgtttgcaacatatgacaaatctgaaacagaaacagccctgttcatacccattttagatttaacagttggaaaggtggagaacgcagctgaaggtagttggaatttccattcaacaattggaactgtgacaccttcgtgaactctaatatctcctatggtgtaagcacgataagcacgacgaatatagacttgagcagctgcagcagtcacaactgggtcttgatgggttaggaattgaagtaaaacatcgaacacaacgtaattagaatcgatcaagtccttcaagatattcaaatctggttcagagcgctttggattggatgagccataggcaaccttcacaacagaggattttaagatatgttcaatttgttcagttctttccttgaccgaaggtaaagcgccttgaatcaaaatttctcttgcttgtagagcgaccttagcggtagccttagattctagttcaacaatatgttgtagaggagtagagaaaatggcagaaactttagaagataacttgcacaatggttgataatgtttcaagatagctaggatcaggttattcttcgctgaaactttcgaatgagacaaaacagttagcgcaactttatctagatctttagggttttcatcacgcaatttcagaatgatattttcctcacgaacatttggaccattgaataacttttcaacttcgtaatattcttccaagaaatggacaaatatagaatgttcatgggcttctaacccgttagagtacttatgagcaatatccgccaatggttccacgacggcgcccagcaatttgtcggggttgtattcaggattcttcacggccatatcaatcaatttacttaattgtctagctgggaaaacagcaccacgtctcaaagaacgtgcaactaactcttccatttgttcatctagcttagcaggcaatcttgaatgtaaagcagagatgtgtagtttccattctgagtaaggcagttttggatttctcaaaacctctatcaattgttgcaaggaagcgttcataataacttggttgtcataacccttcaaaatgttttccaaagtagacactaatgacttgaatttataggcaggtttggttccttcgataactggagaaccaaaatctggcagcataccttcaaatggtagagcgtgcttgaccttggatggatcgtcaagagtcataatagccatgatatcacctgcaacaatggtagaaccaggttgctttaataactggacgataccattttcttgagaaaccaaaggcatttgcattttcataacttcaatttctgcatatggttggcccttgataatgtgttcaccattttccaccaagaatttaaccaatttaccaggggatggagtacgcaactgggttggatcgttttcaacttccaacaaagtagtcatagagtcaacggataatcttgtagcagcaacttcttctttccaatagatggtatgcgatttaccgcctatggcaatcaaaagaccaccatcagatagttgacgcagtatgatatcacatttagaaccattgataaataatgtgtaacggtcattaccggatttagctacggtgaacttgtatcttttaccctcatggataaaatctacagggaacatagtttgcagtaggtctttagatagaacttgtcccttttgtaaggattcgatatacttgtggcgggcttcttcagatgctaagaaagcctttgtagcggcaccgcaaatgacggcaagagttggatcaggcttttcagcggtcattttatgagtaatcaaatcgtccaaccaaccggtggtaatagtgttatcctcgaaatcttcagtttccaaaagtttgatcaagtattccacagtagttctgaaatcacccctaatggacaattccttcagggcaacaaccatgtgtttcctggaagcttgtctattttcaccaaaagcaaaaatatggccgaactgagagtccgaaaaggagtgaatattaccattgttacccacggagaagtaaccccaaacattagaggaagaacggaagtttagttcatgcaaagtaccacccgatggcttgaatccatcgtttggatcttctgatgtgatacgacaagcggtacaatgaccctttggaataggtcttctttgtttcttggtggcatcttgagttttgaattcgaaatcgatttctgaggcagaatgaggattcataccatataaagttctaatgtcacttattctatgcatagggatacccatagcgatttgtaattgagctgcaggtaagttaacaccggagaccatttccgttgttggatgctcgacttgtaatcttgggttcaattctaaaaagtagaattttccatcatcatgagaatatagatactccacggtaccggcagagacataaccgactagtttccccagtctgacggcagccttttccatctcgtgaaatgtttcagccttggcaattgtaactggtgcttcttcgataattttttgatgacgtctctgaacggaacagtctctaccgaacaaggaaatatttgtaccgtactgatctgctagcagttgaacttccaagtgacgcgctctaccggccaacttcatgatgaaaatgggggagcctggaatttcgttggctgcctggtggtataaagcgatgaaatcttcttcacgttcaacttgtctgatacctttaccaccaccaccttcggatgccttaatcatgacaggaaaaccaatacgcttggccttttgtaaaccatcttcaggagaggtacaacaacccttttgatagatgtcatcgtcgacagagaccagaccggttttctcgtccacgtgaacggtgtcaacaccggtaccagaccatggaatacatgggactttagcactttgagcgacaatggtagaggagattttatcacctaaagacctcatggcgttacctggaggcccaataaagatgactttcctcttagactgggacaatttttcaggcaatagtggattctcggaggcgtgaccccagccagcccatacggcgtctacgtctgctctttcggcgatgtctacgatcaagtctacgttagcgtagttgttattattagtaccacctggcacttcaatgtattgatcggccatacggatatattctgcgttggcctccagatcttctggggtggccatggcgacgaattggacggttctgtcatcgccgaacgtctcgtatgcccattttctgacggatctaatttctttcacggcggcaataccattatttgctatcaggatcttggatatgaccgtgtgaccaccgtgactcttaacaaagtcccttaacggggactcctctagtttatctactgtattgaggccaatgaaatgacctggaagttctgtatgtctttctgagtagtttgtaatttcgtactccatcttctgtggagaagactcgaataagctttcttcgctcatgttttcttgccccctatttgcatgaaaatacaatagatgaatagtcattcgctataaaattatttatttgaatatcttatttcctatcagactaagcatagaaatccaatcactaggattattaactaataagtattgtgagtattgaaaaaaagttctgaatctgggggaacacttcactatatattaatatgttggaaccccctttatattatttaaaataatataataatataatttttaataaagggcggcttctcctatgtcggagctcgtttaaacgagctcgctcccccgccgtcgttcaatgtgaatggataagaggctcgtgggattgacgtgagggggcagggatggctatatttctgggagaattaaccgatcgacgtgcaagcggacatttattttaaattcgataatttttgcaaaaacatttcgacatatttatttattttattattatgacatgtttttttggggtacagtctatgcctcgggcatccaagcagcaagcgcgttacgccgtgggtcgatgtttgatgttatggagcagcaacgatgttacgcagcagggcagtcgccctaaaacaaagttaaacatcatgggggaagcggtgatcgccgaagtatcgactcaactatcagaggtagttggcgtcatcgagcgccatctcgaaccgacgttgctggccgtacatttgtacggctccgcagtggatggcggcctgaagccacacagtgatattgatttgctggttacggtgaccgtaaggcttgatgaaacaacgcggcgagctttgatcaacgaccttttggaaacttcggcttcccctggagagagcgagattctccgcgctgtagaagtcaccattgttgtgcacgacgacatcattccgtggcgttatccagctaagcgcgaactgcaatttggagaatggcagcgcaatgacattcttgcaggtatcttcgagccagccacgatcgacattgatctggctatcttgctgacaaaagcaagagaacatagcgttgccttggtaggtccagcggcggaggaactctttgatccggttcctgaacaggatctatttgaggcgctaaatgaaaccttaacgctatggaactcgccgcccgactgggctggcgatgagcgaaatgtagtgcttacgttgtcccgcatttggtacagcgcagtaaccggcaaaatcgcgccgaaggatgtcgctgccgactgggcaatggagcgcctgccggcccagtatcagcccgtcatacttgaagctagacaggcttatcttggacaagaagaagatcgcttggcctcgcgcgcagatcagttggaagaatttgtccactacgtgaaaggcgagatcaccaaggtagtcggcaaataaacccaaataatgttttaaaattttaaaaataatgtaggaggaaaaattatggtgagtaaaggtgaagagttgattaaagagaacatgcatatgaagttatacatggagggaactgtcaataatcaccactttaagtgtacatcagagggtgagggaaagccatacgagggaacccaaactatgagaatcaaagtagtggagggaggtcctcttccatttgcttttgatatactagcaacaagtttcatgtatggttccaggaccttcattaaccatactcagggaatccctgacttctttaaacagtcttttcctgaaggttttacatgggagagggttaccacttacgaggacggtggagtcttgacagcaacccaggacacttcattacaagatggatgcctaatatacaatgtgaaaattaggggtgtgaatttccctagtaacggaccagttatgcagaagaaaacactaggttgggaagctaatactgaaatgttgtaccctgccgacggaggtttagaaggtagatccgacatggcccttaagctagtcggaggtggacacttgatctgtaactttaaaaccacatataggtctaagaagccagcaaagaatctaaaaatgcctggtgtttactatgtggaccatagactagaaaggataaaagaagcagacaaagaaacttacgtggagcaacatgaggtcgccgtcgctaggtattgcgacttaccttccaagctaggtcacaaattgaactccggactctagggatccaaacagtagacattagcagataaattagcaggaaataaagaaggataaggagaaagaactcaagtaattatccttcgttctcttaattgaattgcaattaaactcggcccaatcttttactaaaaggattgagccgaatacaacaaagattctattgcatatattttgactaagtatatacttacctagatatacaagatttgaaatacaaaatctagagcatgcgcgatcgcgctgattgacgcgtcagtacaatctgctctgatggatccgggcccataacttcgtataaagtatcctatacgaagttatagatcctgttaaacagagaagctgggggatatcagctggatggcaaataatgattttattttgactgatagtgacctgttcgttgcaacaaattgataagcaatgctttcttataatgccaactttgtacaagaaagctgggtgaattcgtcttctccccccgccacgatcgaacgggaatggataagaggcttgtgggattgacgtgatagggtagggttggctatactgctggtggcgaactccaggctaataatctgaagcgcggaagttgtagggaggatccttctttcatgcatactccactgttttagagctagaaatagcaagttaaaataaggctagtccgttatcaacttgaaaaagtggcaccgagtcggtgcttttttttctagaggggtctcttcgatagactaagtggatcccgtgatagaaaaaggtctaataacaaagaccagaaatagaaagatcaaaaatcagttacgaaaatgcagtaattcttctttggtcaaacgattgattgcaattgaactcggctcaatctgaaaaagattgagccgagttcaaatagattttgatacgatcatgagacttgacaaatcgggattcctctactctatatatttagaaggtataaaggtatcctccaataaataaatacaaccaagatctgacggtatcgaaccccagagtcatcgagcctgcttttttgtacaaagttggcattataaaaaagcattgctcatcaatttgttgcaacgaacaggtcactatcagtcaaaataaaatcattatttggggcccgagcttaagcctaggtcgactttcacagtttccattctgaaatgttctctgtactataataaatagtaagtgaatcaacttactactaaaaaaattagtagacttcctcttcggaatagaaatagcctatttctacatagggaaagtcgtgtgcaatgaaaaatgcaagcacgatttggggagaggttttttctctattgtaacaaggaataattatctactccatccgactagttccgggttcgagtcccgggcaacccatatggaaactagaaaggagcaatctgagttttgatttttcactcacttcatttacaaaattttttggtttggtaaattttgttgtatggatatacaactgtcggggctggcttggttgacattggtatatagtctatattatactgttaaataacaagccttctattatctttctagttaatacgtgtgcttgggagtccttgcaatttgaataaaccaagatcttaccatggacaagaagtactcgatcgggctggccatcggaacaaattctgtaggctgggctgtaataaccgatgagtacaaggtgccctctaaaaaatttaaggtccttggcaatacggatagacattccataaagaagaatcttatcggtgcgctgctctttgacagcggcgagaccgcggaggcgacccggttgaaacgcaccgcgagacgccgttacacaaggcgtaagaatagaatctgttatctccaggagatattctctaatgaaatggcgaaggtagacgattccttctttcaccgtctggaggaaagttttctcgttgaggaagataagaaacatgaaagacacccgatcttcggaaacattgtcgacgaggttgcttatcatgaaaagtaccctaccatctaccatcttagaaagaaacttgttgacagcacggataaggctgatctcaggctgatatacctggctctggcacatatgattaagttcagagggcatttccttatcgaaggcgacctgaatccagataattcagatgtagacaagctcttcattcaacttgtgcagacttataatcagctcttcgaagaaaatccaataaacgcgtcgggtgtagacgcaaaggccatactgtccgctaggctttctaagtcacgtagacttgagaatctcattgcccaactccccggcgagaagaagaacggcttgtttggaaatctgatagcgctgtccctgggtcttacaccaaatttcaagagtaatttcgatttggcagaagatgctaagttgcagctcagtaaagacacctacgatgacgatcttgataatttgttggctcagattggcgatcagtatgcagatcttttcttggccgctaagaatttgtctgatgcaattctgcttagcgacattttgagggttaatacagaaatcaccaaggcacccttgtcggcgtcaatgataaagaggtatgatgagcaccaccaagacctgacgctcctcaaggctcttgttcggcagcaattgccggagaagtacaaagagatcttcttcgaccagtctaagaacggatatgcgggctacatagacggtggagcgagtcaggaggaattctacaagttcataaagcccattctcgagaagatggatggtacggaagaactgcttgtgaaacttaacagagaagatcttttgcggaagcagagaactttcgacaacggaagtataccacaccagatacatctcggagagcttcatgctattctcagaagacaagaggatttctaccctttcttgaaggataacagagaaaagatagagaagatcctcacgtttaggatcccttactacgtaggtcctcttgctcgcggcaatagtaggttcgcctggatgacccgcaagtctgaagaaactatcaccccttggaatttcgaagaggttgtagacaaaggtgcttcagcacagagtttcattgagaggatgaccaacttcgacaagaacctccccaacgaaaaggtcctgcctaagcacagcctcctctacgaatactttactgtctataatgagcttacaaaagttaagtacgtgacagagggaatgcggaagcccgcattcctttccggagaacaaaagaaggcgatcgtggatcttctcttcaagacgaaccgcaaggtgacggttaaacagttgaaggaagattacttcaagaagatagaatgttttgatagcgtggaaatcagcggcgtcgaagataggttcaacgcttccctgggaacgtaccacgatctcctcaagattatcaaagataaggactttcttgataacgaagagaatgaggacatcttggaagacattgttctgacgctcaccctgttcgaagatcgcgagatgattgaggaacgcttgaagacctacgcacacctgttcgatgacaaggttatgaagcaacttaaacggcgccggtatacgggctggggacggctttcgcggaagctgataaatggaatccgtgacaagcagtctggcaagacaatactcgacttcttgaagtcggatggttttgccaatagaaattttatgcaactcattcatgatgactcgcttacttttaaggaggacatccagaaggcccaggtatcaggacagggtgactctttgcacgaacacatcgcgaacctggcgggctcccccgcgattaagaagggaattttgcagactgtcaaggtggtcgatgaactcgtgaaggttatgggacgtcataagccggaaaatattgtgattgagatggctcgcgagaatcaaacaacacagaagggccaaaagaacagtagagaacgcatgaagcgcatcgaagagggcatcaaagagctgggcagtcagatccttaaagaacatccagtcgagaatacacagcttcagaacgaaaagctgtacctttattaccttcaaaatgggcgtgatatgtatgtggatcaggaactcgatatcaataggctgagtgactatgatgtcgaccatatcgtcccgcaaagtttcctcaaggacgacagtatagacaacaaagttctcacacggtcagataagaatcgcggcaagagcgataatgtaccgtcggaggaggtagtcaagaagatgaagaattactggcgccagttgctcaacgccaagctcatcactcagaggaaatttgacaaccttacgaaagccgagcggggcggactctctgaactggacaaggccggtttcataaagcgccagctcgttgagacacgtcaaattactaagcacgtcgctcaaatattggattcccgcatgaatactaagtacgatgagaatgataagctcatacgtgaagttaaggtcattactctcaagtccaagcttgtatcggacttccgtaaggacttccaattctacaaggtccgggaaatcaataattatcaccatgcccatgacgcttatctgaacgcggtcgtgggcacggcactcattaagaaatacccaaaacttgagtcagaatttgtttacggggactataaagtttatgacgtgcggaagatgatagcgaagtcggaacaagagataggaaaggcgactgcaaagtactttttttactccaacataatgaatttctttaagaccgaaataacccttgcaaacggtgaaatcagaaagcggcctctgattgaaacaaatggcgagacgggcgagatcgtctgggacaaggggagggacttcgcaacggttcgcaaggtccttagcatgccgcaagtaaatatagttaagaagacggaagttcagaccggcggctttagtaaagaaagcatacttcctaaaaggaattccgacaaactgatagcgcgcaagaaggactgggatccaaagaagtatggaggatttgactccccaaccgttgcttatagcgtgttggtagtagccaaggtggaaaagggtaagtctaagaaattgaagtcggtgaaggagttgttggggataactataatggagcggagttcgttcgagaagaacccaattgactttctcgaagccaaaggctacaaggaggtcaagaaggacctgattattaagttgccaaagtactcgctcttcgaactcgagaacgggagaaagcgtatgctggcgtcggcgggcgagctgcagaaaggaaacgagctggctttgccatcgaaatacgtaaatttcctgtacctcgcctcacattatgagaagcttaaagggtctccagaagacaatgaacagaagcagctgtttgttgaacagcacaagcactacttggacgagattatagaacaaatctccgagttctctaaacgggttatccttgcagacgccaatttggataaggtcctctcggcttataataagcatagagataagccaatccgggagcaggctgaaaatatcatacacctctttacgttgactaatttgggtgcgccagcggcattcaagtacttcgatacaacaatcgatcgtaagcgctacacaagcactaaggaagtcctggacgcgacgctgatacaccagtccattactggactgtatgaaaccagaatagatcttagccagctcggcggtgattagcccgccggcgcatcgtcggctacagcctcggtggggaataattaattaaggcttttctgctaacatatagcaatttttgaagaaaggaaagctagaaatacccaatatcttgctgaagcaagatattgggtatttcttttttttttattttgaatctttctattctgaattcagttaacgacgagatttagtatcctttcttgcactttcataactcgtgaaatgccgagttggtacgaattcccccaatttgcgacctaccataggatttgttatgtaaataggtatatgttcctttccattatgaatcgcgattgtatggccaaccattgcgggtagaatgctagatgcccgggaccacgttactattgtttctttctcctccttcatattgagcttttctatttttgccaataaatgatgcggccacgaagcggccgcgtagcgtttataggatataacttcgtataggatactttatacgaagttatgggcccggtagtgttctgtcatgatgcggcgcgccctcggggggatatagctcagttggtagagctccgctcttgcaattgggtcgttgcgattacgggttggctgtctaattgtccaggcggtaatggtagtatcttgtacctgaaccggtggctcactttttctaagtaatggggaagaggactgaaacatgccactgaaagactctactgagacaaaaagatgggctgtcaaaaaggtagaggaggtaggatgggcagttggtcagatctagtatggatcgtacatggacgatagttggagtcggcggctctcctaggcttccctcatctgggatccctggggaagaggatcaagtgtggcccttgcgaatagcttgatgcactatctcccttcaaccctttgagcgaaatgtggcaaaaggaaggaaaatccatggaccgaccccattatctccaccccgtaggaactacgagatcaccccaaggacgccttcggcgtccaggggtcacggaccgaccatagaccctgttcaataagtggaacacattagccgtccgctctccggttgggcagtaagggtcggagaagggcaatcactcgttcttaaaaccagcattcttaagtttaagatcaaagagtcgggcggaaaaaggggagagctccccgttcctggttctcctgtagctggattccccggaaccacaagaatccttagaatgggattccaactcagcaccttttgttttgagattttgagaagagttgctctttggagagcacagtacgatgaaagttgtaagctgtgttcgggggggagttattgtctatcgttggcctctatggtagaacccgtcggggaggcctgagaggcggtggtttaccctgtggcggatgtcagcggttcgagtccgcttatctccagcccgtgaacttagcggatactatgatagcaccgaattttgccaattcggcagttcgatctatgatttcgcattcatggacgttgataagatccttccatttagtagcaccttaggatggcatagccttaacgttaatggcgaggttcaaaagaggaaaggcttgcggtggatacctaggtacccagagacgaggaagggcgtagcaagcgacgaaatgcttcggggagttgaaaataagcatagatccggagattcccaaataggtcaaccttttgaactgcctgctgaatccatgagcaggcaagagacaacctggcgaactgaaacatcttagtagccagaggaaaagaaagcaaaagcgattcccgtagtagcggcgagcgaaatgggagcagcctaaaccgtgaaaacggggttgtgggagagcaatacaagcgttgtgctgctaggcgaagcggttgagtgccgcaccctagatggctaaagtccagtagccgaaagcatcactagcttacgctctgacccgagtagcatggggcacgtggaatcccgtgtgaatcagcaaggaccaccttgcaaggctaaatactcctgggtgaccgatagcgaagtagtaccgtgagggaaaggtgaaaagaacccccagtgggtagtgaaatagaacgtgaaaccgtgctgagctcccaagcagtgggaggggaaagtgatctctgaccgcgtgcctgttgaagaatgagccggcgactcataggcagtggcttggttaa

SEQ ID NO: 7 - DNA, 7678 bp, Artificial Sequence
  full-sequence of pNC
  gene (2351)..(3142): aadA
  gene (3191)..(3913): TagRFP
ctttcctgcgttatcccctgattctgtggataaccgtattaccgcctttgagtgagctgataccgctcgccgcagccgaacgaccgagcgcagcgagtcagtgagcgaggaagcggaagagcgcccaatacgcaaaccgcctctccccgcgcgttggccgattcattaatgcagctggcacgacaggtttcccgactggaaagcgggcagtgagcgcaacgcaattaatacgcgtaccgctagccaggaagagtttgtagaaacgcaaaaaggccatccgtcaggatggccttctgcttagtttgatgcctggcagtttatggcgggcgtcctgcccgccaccctccgggccgttgcttcacaacgttcaaatccgctcccggcggatttgtcctactcaggagagcgttcaccgacaaacaacagataaaacgaaaggcccagtcttccgactgagcctttcgttttatttgatgcctggcagttccctactctcgcgttaacgctagcatggatgttttcccagtcacgacgttgtaaaacgacggccagtcttaagctcgggccccaaataatgattttattttgactgatagtgacctgttcgttgcaacaaattgatgagcaatgcttttttataatgccaactttgtacaaaaaagcaggcttgaagccggaatcgctagtaatcgccggtcagccatacggcggtgaattcgttcccgggccttgtacacaccgcccgtcacactatgggagctggccatgcccgaagtcgttaccttaaccgcaaggaggggggtgccgaaggcagggctagtgactggagtgaagtcgtaacaaggtagccgtactggaaggtgcggctggatcacctccttttcagggagagctaatgcttcttgggtatttaggtttgacacagcttcacacccaaaaagaagggagctacgtctgagttaaacttggaggtggaagccttctttcgtttctcgacggtgaagtaagaccaaacccatgagcttattatcctaggtcggaacaagttgataggatccccttttacgcccccatgtccctctcgtgtggcggcagggaggcgtaaaaaggaaagagagagatggggtttctctcgcttttggcttggcatagcgggcccccagcaggaggcccgcacgacgggctattagctcagtggtagagcgcgcccctgataattgcgtcgttgtgcctgggctgtgagggctctcagccacatggatagttcaatgtgctcatcagcgcctgaccctgagatgtggatcatccaaggcacattagcatggcgtactcctcctgttcgaaccggggtttgaaaccaaacttctcctcaggaggatagatggggcgattcaggtgagatccaatgtagatccaactttctattcactcgtgggatccgggcggtccggaggggaccactatggctcctctcttctcgagaatccatacatcccttatcagtgtatggacagctatctctcgagcgcaggtttaggttcggcctcaatgggaaaataaaatggagcacctaacaacgtatcttcacagaccaagaactacgagatcacccctttcattctggggtgacggagggatcgtaccgttcgagcctttttttcatgttatctatctcttgactcgaaatgggagcaggtttgaaaaaggatcttagagtgtctagggttaggccagtagggtctcttaacgccctcttttttcttctcatcgaagttatttcacaaatacttcctatggtaaggaagagggggggaacaagcacacttggagagcgcagtacaacggagagttgtatgctgcgttcgggaaggatgaatcgctcccgaaaaggaatctattgattctctcccaattggttggaccataggtgcgatgatttacttcacgggcgaggtctctggttcaaatccaggatggcccagctgcgccaaggaaaagaatataagaaggatctgactccttcatgcatggagctcgctcccccgccgtcgttcaatgtgaatggataagaggctcgtgggattgacgtgagggggcagggatggctatatttctgggagaattaaccgatcgacgtgcaagcggacatttattttaaattcgataatttttgcaaaaacatttcgacatatttatttattttattattatgacatgtttttttggggtacagtctatgcctcgggcatccaagcagcaagcgcgttacgccgtgggtcgatgtttgatgttatggagcagcaacgatgttacgcagcagggcagtcgccctaaaacaaagttaaacatcatgggggaagcggtgatcgccgaagtatcgactcaactatcagaggtagttggcgtcatcgagcgccatctcgaaccgacgttgctggccgtacatttgtacggctccgcagtggatggcggcctgaagccacacagtgatattgatttgctggttacggtgaccgtaaggcttgatgaaacaacgcggcgagctttgatcaacgaccttttggaaacttcggcttcccctggagagagcgagattctccgcgctgtagaagtcaccattgttgtgcacgacgacatcattccgtggcgttatccagctaagcgcgaactgcaatttggagaatggcagcgcaatgacattcttgcaggtatcttcgagccagccacgatcgacattgatctggctatcttgctgacaaaagcaagagaacatagcgttgccttggtaggtccagcggcggaggaactctttgatccggttcctgaacaggatctatttgaggcgctaaatgaaaccttaacgctatggaactcgccgcccgactgggctggcgatgagcgaaatgtagtgcttacgttgtcccgcatttggtacagcgcagtaaccggcaaaatcgcgccgaaggatgtcgctgccgactgggcaatggagcgcctgccggcccagtatcagcccgtcatacttgaagctagacaggcttatcttggacaagaagaagatcgcttggcctcgcgcgcagatcagttggaagaatttgtccactacgtgaaaggcgagatcaccaaggtagtcggcaaataaacccaaataatgttttaaaattttaaaaataatgtaggaggaaaaattatggtgagtaaaggtgaagagttgattaaagagaacatgcatatgaagttatacatggagggaactgtcaataatcaccactttaagtgtacatcagagggtgagggaaagccatacgagggaacccaaactatgagaatcaaagtagtggagggaggtcctcttccatttgcttttgatatactagcaacaagtttcatgtatggttccaggaccttcattaaccatactcagggaatccctgacttctttaaacagtcttttcctgaaggttttacatgggagagggttaccacttacgaggacggtggagtcttgacagcaacccaggacacttcattacaagatggatgcctaatatacaatgtgaaaattaggggtgtgaatttccctagtaacggaccagttatgcagaagaaaacactaggttgggaagctaatactgaaatgttgtaccctgccgacggaggtttagaaggtagatccgacatggcccttaagctagtcggaggtggacacttgatctgtaactttaaaaccacatataggtctaagaagccagcaaagaatctaaaaatgcctggtgtttactatgtggaccatagactagaaaggataaaagaagcagacaaagaaacttacgtggagcaacatgaggtcgccgtcgctaggtattgcgacttaccttccaagctaggtcacaaattgaactccggactctagggatccaaacagtagacattagcagataaattagcaggaaataaagaaggataaggagaaagaactcaagtaattatccttcgttctcttaattgaattgcaattaaactcggcccaatcttttactaaaaggattgagccgaatacaacaaagattctattgcatatattttgactaagtatatacttacctagatatacaagatttgaaatacaaaatctagagcatgcctccacttggctcgggggatatagctcagttggtagagctccgctcttgcaattgggtcgttgcgattacgggttgggtgtctaattgtccaggcggtaatgatagtatcttgtacctgaaccggtggctcactttttctaagtaatggggaaaaggaccgaaacatgccactgaaagactctactgagacaaagatgggctgtcaagaacgtagaggaggtaggatggtcagttggtcagatctagtatggatcgtacatggacggtagttggagtcggcggctctcctagggttccctcgtctgggattgatccctggggaagaggatcaagttggcccttgcgaacagcttgatgcactatctcccttcaaccctttgagcgaaatgcggcaaaaggaaggaaaatccatggaccgaccccatcgtctccaccccgtaggaactacgagatcaccccaaggacgccttcggtatccaggggtcgcggaccgaccatagaaccctgttcaataagtggaatgcattagctgtccgctcgcaggttgggcagtaagggtcggagaagggcaatcactcattcttaaaaccagcattcgaaagagttggggcggaaaagggggggaaagctctccgttcctggttctcctgtagctggatcctctagaaccacaagaatccttagttggaatgggattccagctcatcaccttttgagattttgagaagagttgctctttggagagcacagtacgatgaaagttgtaagctgtgttcgggggggagttcttgtctatcgttggcctctatggtagaatcagtcaggggcctgataggcggtggtttaccctgtggcggatgtcagcggttcgagtccgcttatctccaactcgtgaacttagccgatacaaagctatatgatagcacccaatttttccgattcggcagttcgatctatgatttttcattcatggacgttgataagatctttccatttagcagcaccttaggatggcatagccttaaagttaagggcgaggttcaaacgaggaaaggcttacggtggatacctaggcacccagagacgaggaagggcgtagtaagcgacgaaatgcttcggggagttgaaaataagcgtagatccggagattcccgaataggttaaccttttgaactgctgctgaatccatgggcaggcaagagacaacctggcgaactgaaacatcttagtagccagaggaaaagaaagcaaaagcgattcccgtagtagcggcgagcgaaatgggagcagcctaaaccgtgaaaacggggttgtgggagagcaaaaaaagcgtcgtgctgctaggcgaagcggtggagtgccgcaccctagatggcgagagtccagtagccgaaagcatcactagcttatgctctgacccgagtagcatggggcacgtggaatcccgtgtgaatcagcaaggaccaccttgcaaggctaaatactcctgggtgaccgatagcgaagtagtaccgtgagggaagggtgaaaagaacccccatcggggagtgaaatagaacatgaaaccgtaagctcccaagcagtgggaggagccctgggctctgaccgcgtgcctgttgaagaatgagccggcgactcataggcagtggcttggttaacccagctttcttgtacaaagttggcattataagaaagcattgcttatcaatttgttgcaacgaacaggtcactatcagtcaaaataaaatcattatttgccatccagctgatatcccctatagtgagtcgtattacatggtcatagctgtttcctggcagctctggcccgtgtctcaaaatctctgatgttacattgcacaagataaaaatatatcatcatgaacaataaaactgtctgcttacataaacagtaatacaaggggtgttatgagccatattcaacgggaaacgtcgaggccgcgattaaattccaacatggatgctgatttatatgggtataaatgggctcgcgataatgtcgggcaatcaggtgcgacaatctatcgcttgtatgggaagcccgatgcgccagagttgtttctgaaacatggcaaaggtagcgttgccaatgatgttacagatgagatggtcagactaaactggctgacggaatttatgcctcttccgaccatcaagcattttatccgtactcctgatgatgcatggttactcaccactgcgatccccggaaaaacagcattccaggtattagaagaatatcctgattcaggtgaaaatattgttgatgcgctggcagtgttcctgcgccggttgcattcgattcctgtttgtaattgtccttttaacagcgatcgcgtatttcgtctcgctcaggcgcaatcacgaatgaataacggtttggttgatgcgagtgattttgatgacgagcgtaatggctggcctgttgaacaagtctggaaagaaatgcataaacttttgccattctcaccggattcagtcgtcactcatggtgatttctcacttgataaccttatttttgacgaggggaaattaataggttgtattgatgttggacgagtcggaatcgcagaccgataccaggatcttgccatcctatggaactgcctcggtgagttttctccttcattacagaaacggctttttcaaaaatatggtattgataatcctgatatgaataaattgcagtttcatttgatgctcgatgagtttttctaatcagaattggttaattggttgtaacactggcagagcattacgctgacttgacgggacggcgcaagctcatgaccaaaatcccttaacgtgagttacgcgtcgttccactgagcgtcagaccccgtagaaaagatcaaaggatcttcttgagatcctttttttctgcgcgtaatctgctgcttgcaaacaaaaaaaccaccgctaccagcggtggtttgtttgccggatcaagagctaccaactctttttccgaaggtaactggcttcagcagagcgcagataccaaatactgttcttctagtgtagccgtagttaggccaccacttcaagaactctgtagcaccgcctacatacctcgctctgctaatcctgttaccagtggctgctgccagtggcgataagtcgtgtcttaccgggttggactcaagacgatagttaccggataaggcgcagcggtcgggctgaacggggggttcgtgcacacagcccagcttggagcgaacgacctacaccgaactgagatacctacagcgtgagctatgagaaagcgccacgcttcccgaagggagaaaggcggacaggtatccggtaagcggcagggtcggaacaggagagcgcacgagggagcttccagggggaaacgcctggtatctttatagtcctgtcgggtttcgccacctctgacttgagcgtcgatttttgtgatgctcgtcaggggggcggagcctatggaaaaacgccagcaacgcggcctttttacggttcctggccttttgctggccttttgctcacatgtt

SEQ ID NO: 8 - DNA, 20 bp, Artificial Sequence
  PCR Primer
cacttcaatgtattgatcgg

SEQ ID NO: 9 - DNA, 26 bp, Artificial Sequence
  PCR Primer
tcgagtcttctccacagaagatggag

SEQ ID NO: 10 - DNA, 30 bp, Artificial Sequence
  PCR Primer
atgctgaagatcagttgggtgcacgagtgg

SEQ ID NO: 11 - DNA, 30 bp, Artificial Sequence
  PCR Primer
ttaatcagtgaggcacctatctcagcgatc

SEQ ID NO: 12 - DNA, 30 bp, Artificial Sequence
  PCR Primer
atcggagttatttcccaaggacttgccatg

SEQ ID NO: 13 - DNA, 30 bp, Artificial Sequence
  PCR Primer
ccgccgactccaactatcgtccatgtacga

SEQ ID NO: 14 - DNA, 7679 bp, Artificial Sequence
  full-sequence of pKK4
  misc_feature (669)..(2030): AtCp1_flanking
  gene (2187)..(2960): AtPGP1(cDNA, d39)
  gene (3195)..(3914): mClover
  misc_feature (4146)..(5802): AtCp1_flanking
ctttcctgcgttatcccctgattctgtggataaccgtattaccgcctttgagtgagctgataccgctcgccgcagccgaacgaccgagcgcagcgagtcagtgagcgaggaagcggaagagcgcccaatacgcaaaccgcctctccccgcgcgttggccgattcattaatgcagctggcacgacaggtttcccgactggaaagcgggcagtgagcgcaacgcaattaatacgcgtaccgctagccaggaagagtttgtagaaacgcaaaaaggccatccgtcaggatggccttctgcttagtttgatgcctggcagtttatggcgggcgtcctgcccgccaccctccgggccgttgcttcacaacgttcaaatccgctcccggcggatttgtcctactcaggagagcgttcaccgacaaacaacagataaaacgaaaggcccagtcttccgactgagcctttcgttttatttgatgcctggcagttccctactctcgcgttaacgctagcatggatgttttcccagtcacgacgttgtaaaacgacggccagtcttaagctcgggccccaaataatgattttattttgactgatagtgacctgttcgttgcaacaaattgatgagcaatgcttttttataatgccaactttgtacaaaaaagcaggcttgaagccggaatcgctagtaatcgccggtcagccatacggcggtgaattcgttcccgggccttgtacacaccgcccgtcacactatgggagctggccatgcccgaagtcgttaccttaaccgcaaggaggggggtgccgaaggcagggctagtgactggagtgaagtcgtaacaaggtagccgtactggaaggtgcggctggatcacctccttttcagggagagctaatgcttcttgggtatttaggtttgacacagcttcacacccaaaaagaagggagctacgtctgagttaaacttggaggtggaagccttctttcgtttctcgacggtgaagtaagaccaaacccatgagcttattatcctaggtcggaacaagttgataggatccccttttacgcccccatgtccctctcgtgtggcggcagggaggcgtaaaaaggaaagagagagatggggtttctctcgcttttggcttggcatagcgggcccccagcaggaggcccgcacgacgggctattagctcagtggtagagcgcgcccctgataattgcgtcgttgtgcctgggctgtgagggctctcagccacatggatagttcaatgtgctcatcagcgcctgaccctgagatgtggatcatccaaggcacattagcatggcgtactcctcctgttcgaaccggggtttgaaaccaaacttctcctcaggaggatagatggggcgattcaggtgagatccaatgtagatccaactttctattcactcgtgggatccgggcggtccggaggggaccactatggctcctctcttctcgagaatccatacatcccttatcagtgtatggacagctatctctcgagcgcaggtttaggttcggcctcaatgggaaaataaaatggagcacctaacaacgtatcttcacagaccaagaactacgagatcacccctttcattctggggtgacggagggatcgtaccgttcgagcctttttttcatgttatctatctcttgactcgaaatgggagcaggtttgaaaaaggatcttagagtgtctagggttaggccagtagggtctcttaacgccctcttttttcttctcatcgaagttatttcacaaatacttcctatggtaaggaagagggggggaacaagcacacttggagagcgcagtacaacggagagttgtatgctgcgttcgggaaggatgaatcgctcccgaaaaggaatctattgattctctcccaattggttggaccataggtgcgatgatttacttcacgggcgaggtctctggttcaaatccaggatggcccagctgcgccaaggaaaagaatataagaaggatctgactccttcatgcatggagctcgctcccccgccgtcgttcaatgtgaatggataagaggctcgtgggattgacgtgagggggcagggatggctatatttctgggagggagaccacaacggtttcccactagaaataattttgtttaactttaagaaggagatatatcatatgtactcctcccgtacatctctaaggtttccgattcaaatatctcgccaccaacaccgtctatcctacttttcttcatcctcttcgtcggagcaaagcagaccaacttcctcttcccgaaacagtttcagtggtcacggtcagcttgatagtgatgataattcttcaccgcctccgtcgcaatcatcttccaaagttcttacattgcctaccgtattaacacttggtcgtgtcgccgccgtcccgcttctcgtcgcaaccttttacgttgatagttggtggggaacaactgctacaacaagcattttcattgcagcagccattacagactggcttgacggctatcttgcccgcaagatgaggttaggttctgcgtttggtgcctttttggatccagttgctgataagcttatggttgcagctacattgattttactgtgtacaaaacctatccaagttgctgaattaggaccacttccatggttattgaccgtaccttctattgcaatcattggtagggagattactatgtccgcagtaagagaatgggctgcatctcaaaatggaaagcttttagaggcagttgctgtaaataacttgggcaagtggaaaaccgccacgcagatgacagcactaaccatacttcttgcaagccgagatagcaatgttggatggctcgtagcttcaggtgctggcttgctttatgtatcagcaggactatctgtttggtctttagccgtttatatgaggaagatatggaaagtactaatgaagtagctcgacaattcaatggaagcaatgataaaaaaatacaaatagaaaaggaaagggaggaaatacaaaaaaatagaagagaaaagtcatacaaagttatatacaaatgactacccccctttttgtatttccttaatttatttccttaattgaatttcctcgacagcttaggatcgtttatttacaacggaatggtatacaaagtcaacagatctcaagttgtagggagggatttccatggtgagcaagggcgaggagctgttcaccggggtggtgcccatcctggtcgagctggacggcgacgtaaacggccacaagttcagcgtccgcggcgagggcgagggcgatgccaccaacggcaagctgaccctgaagttcatctgcaccaccggcaagctgcccgtgccctggcccaccctcgtgaccaccttcggctacggcgtggcctgcttcagccgctaccccgaccacatgaagcagcacgacttcttcaagtccgccatgcccgaaggctacgtccaggagcgcaccatctctttcaaggacgacggtacctacaagacccgcgccgaggtgaagttcgagggcgacaccctggtgaaccgcatcgagctgaagggcatcgacttcaaggaggacggcaacatcctggggcacaagctggagtacaacttcaacagccacaacgtctatatcacggccgacaagcagaagaacggcatcaaggctaacttcaagatccgccacaacgttgaggacggcagcgtgcagctcgccgaccactaccagcagaacacccccatcggcgacggccccgtgctgctgcccgacaaccactacctgagcacccagtccaagctgagcaaagaccccaacgagaagcgcgatcacatggtcctgctggagttcgtgaccgccgccgggattacacatggcatggacgagctgtacaagtagggatccaaacagtagacattagcagataaattagcaggaaataaagaaggataaggagaaagaactcaagtaattatccttcgttctcttaattgaattgcaattaaactcggcccaatcttttactaaaaggattgagccgaatacaacaaagattctattgcatatattttgactaagtatatacttacctagatatacaagatttgaaatacaaaatctagagcatgcctccacttggctcgggggatatagctcagttggtagagctccgctcttgcaattgggtcgttgcgattacgggttgggtgtctaattgtccaggcggtaatgatagtatcttgtacctgaaccggtggctcactttttctaagtaatggggaaaaggaccgaaacatgccactgaaagactctactgagacaaagatgggctgtcaagaacgtagaggaggtaggatggtcagttggtcagatctagtatggatcgtacatggacggtagttggagtcggcggctctcctagggttccctcgtctgggattgatccctggggaagaggatcaagttggcccttgcgaacagcttgatgcactatctcccttcaaccctttgagcgaaatgcggcaaaaggaaggaaaatccatggaccgaccccatcgtctccaccccgtaggaactacgagatcaccccaaggacgccttcggtatccaggggtcgcggaccgaccatagaaccctgttcaataagtggaatgcattagctgtccgctcgcaggttgggcagtaagggtcggagaagggcaatcactcattcttaaaaccagcattcgaaagagttggggcggaaaagggggggaaagctctccgttcctggttctcctgtagctggatcctctagaaccacaagaatccttagttggaatgggattccagctcatcaccttttgagattttgagaagagttgctctttggagagcacagtacgatgaaagttgtaagctgtgttcgggggggagttcttgtctatcgttggcctctatggtagaatcagtcaggggcctgataggcggtggtttaccctgtggcggatgtcagcggttcgagtccgcttatctccaactcgtgaacttagccgatacaaagctatatgatagcacccaatttttccgattcggcagttcgatctatgatttttcattcatggacgttgataagatctttccatttagcagcaccttaggatggcatagccttaaagttaagggcgaggttcaaacgaggaaaggcttacggtggatacctaggcacccagagacgaggaagggcgtagtaagcgacgaaatgcttcggggagttgaaaataagcgtagatccggagattcccgaataggttaaccttttgaactgctgctgaatccatgggcaggcaagagacaacctggcgaactgaaacatcttagtagccagaggaaaagaaagcaaaagcgattcccgtagtagcggcgagcgaaatgggagcagcctaaaccgtgaaaacggggttgtgggagagcaaaaaaagcgtcgtgctgctaggcgaagcggtggagtgccgcaccctagatggcgagagtccagtagccgaaagcatcactagcttatgctctgacccgagtagcatggggcacgtggaatcccgtgtgaatcagcaaggaccaccttgcaaggctaaatactcctgggtgaccgatagcgaagtagtaccgtgagggaagggtgaaaagaacccccatcggggagtgaaatagaacatgaaaccgtaagctcccaagcagtgggaggagccctgggctctgaccgcgtgcctgttgaagaatgagccggcgactcataggcagtggcttggttaacccagctttcttgtacaaagttggcattataagaaagcattgcttatcaatttgttgcaacgaacaggtcactatcagtcaaaataaaatcattatttgccatccagctgatatcccctatagtgagtcgtattacatggtcatagctgtttcctggcagctctggcccgtgtctcaaaatctctgatgttacattgcacaagataaaaatatatcatcatgaacaataaaactgtctgcttacataaacagtaatacaaggggtgttatgagccatattcaacgggaaacgtcgaggccgcgattaaattccaacatggatgctgatttatatgggtataaatgggctcgcgataatgtcgggcaatcaggtgcgacaatctatcgcttgtatgggaagcccgatgcgccagagttgtttctgaaacatggcaaaggtagcgttgccaatgatgttacagatgagatggtcagactaaactggctgacggaatttatgcctcttccgaccatcaagcattttatccgtactcctgatgatgcatggttactcaccactgcgatccccggaaaaacagcattccaggtattagaagaatatcctgattcaggtgaaaatattgttgatgcgctggcagtgttcctgcgccggttgcattcgattcctgtttgtaattgtccttttaacagcgatcgcgtatttcgtctcgctcaggcgcaatcacgaatgaataacggtttggttgatgcgagtgattttgatgacgagcgtaatggctggcctgttgaacaagtctggaaagaaatgcataaacttttgccattctcaccggattcagtcgtcactcatggtgatttctcacttgataaccttatttttgacgaggggaaattaataggttgtattgatgttggacgagtcggaatcgcagaccgataccaggatcttgccatcctatggaactgcctcggtgagttttctccttcattacagaaacggctttttcaaaaatatggtattgataatcctgatatgaataaattgcagtttcatttgatgctcgatgagtttttctaatcagaattggttaattggttgtaacactggcagagcattacgctgacttgacgggacggcgcaagctcatgaccaaaatcccttaacgtgagttacgcgtcgttccactgagcgtcagaccccgtagaaaagatcaaaggatcttcttgagatcctttttttctgcgcgtaatctgctgcttgcaaacaaaaaaaccaccgctaccagcggtggtttgtttgccggatcaagagctaccaactctttttccgaaggtaactggcttcagcagagcgcagataccaaatactgttcttctagtgtagccgtagttaggccaccacttcaagaactctgtagcaccgcctacatacctcgctctgctaatcctgttaccagtggctgctgccagtggcgataagtcgtgtcttaccgggttggactcaagacgatagttaccggataaggcgcagcggtcgggctgaacggggggttcgtgcacacagcccagcttggagcgaacgacctacaccgaactgagatacctacagcgtgagctatgagaaagcgccacgcttcccgaagggagaaaggcggacaggtatccggtaagcggcagggtcggaacaggagagcgcacgagggagcttccagggggaaacgcctggtatctttatagtcctgtcgggtttcgccacctctgacttgagcgtcgatttttgtgatgctcgtcaggggggcggagcctatggaaaaacgccagcaacgcggcctttttacggttcctggccttttgctggccttttgctcacatgtt

SEQ ID NO: 15 - DNA, 8876 bp, Artificial Sequence
  full-sequence of pKK5
  misc_feature (669)..(2030): AtCp1_flanking
  gene (2192)..(2965): AtPGP1(cDNA, d39) (complement)
  gene (2969)..(3016): Sac.ACC1 (complement)
  gene (3408)..(4339): aadA
  gene (4389)..(5111): cgfTagRFP
  misc_feature (5343)..(6999): cgfTagRFP
ctttcctgcgttatcccctgattctgtggataaccgtattaccgcctttgagtgagctgataccgctcgccgcagccgaacgaccgagcgcagcgagtcagtgagcgaggaagcggaagagcgcccaatacgcaaaccgcctctccccgcgcgttggccgattcattaatgcagctggcacgacaggtttcccgactggaaagcgggcagtgagcgcaacgcaattaatacgcgtaccgctagccaggaagagtttgtagaaacgcaaaaaggccatccgtcaggatggccttctgcttagtttgatgcctggcagtttatggcgggcgtcctgcccgccaccctccgggccgttgcttcacaacgttcaaatccgctcccggcggatttgtcctactcaggagagcgttcaccgacaaacaacagataaaacgaaaggcccagtcttccgactgagcctttcgttttatttgatgcctggcagttccctactctcgcgttaacgctagcatggatgttttcccagtcacgacgttgtaaaacgacggccagtcttaagctcgggccccaaataatgattttattttgactgatagtgacctgttcgttgcaacaaattgatgagcaatgcttttttataatgccaactttgtacaaaaaagcaggcttgaagccggaatcgctagtaatcgccggtcagccatacggcggtgaattcgttcccgggccttgtacacaccgcccgtcacactatgggagctggccatgcccgaagtcgttaccttaaccgcaaggaggggggtgccgaaggcagggctagtgactggagtgaagtcgtaacaaggtagccgtactggaaggtgcggctggatcacctccttttcagggagagctaatgcttcttgggtatttaggtttgacacagcttcacacccaaaaagaagggagctacgtctgagttaaacttggaggtggaagccttctttcgtttctcgacggtgaagtaagaccaaacccatgagcttattatcctaggtcggaacaagttgataggatccccttttacgcccccatgtccctctcgtgtggcggcagggaggcgtaaaaaggaaagagagagatggggtttctctcgcttttggcttggcatagcgggcccccagcaggaggcccgcacgacgggctattagctcagtggtagagcgcgcccctgataattgcgtcgttgtgcctgggctgtgagggctctcagccacatggatagttcaatgtgctcatcagcgcctgaccctgagatgtggatcatccaaggcacattagcatggcgtactcctcctgttcgaaccggggtttgaaaccaaacttctcctcaggaggatagatggggcgattcaggtgagatccaatgtagatccaactttctattcactcgtgggatccgggcggtccggaggggaccactatggctcctctcttctcgagaatccatacatcccttatcagtgtatggacagctatctctcgagcgcaggtttaggttcggcctcaatgggaaaataaaatggagcacctaacaacgtatcttcacagaccaagaactacgagatcacccctttcattctggggtgacggagggatcgtaccgttcgagcctttttttcatgttatctatctcttgactcgaaatgggagcaggtttgaaaaaggatcttagagtgtctagggttaggccagtagggtctcttaacgccctcttttttcttctcatcgaagttatttcacaaatacttcctatggtaaggaagagggggggaacaagcacacttggagagcgcagtacaacggagagttgtatgctgcgttcgggaaggatgaatcgctcccgaaaaggaatctattgattctctcccaattggttggaccataggtgcgatgatttacttcacgggcgaggtctctggttcaaatccaggatggcccagctgcgccaaggaaaagaatataagaaggatctgactccttcatgcatggtcgacaattcaatggaagcaatgataaaaaaatacaaatagaaaaggaaagggaggaaatacaaaaaaatagaagagaaaagtcatacaaagttatatacaaatgactacccccctttttgtatttccttaatttatttccttaattgaatttcctcgagctacttcattagtactttccatatcttcctcatataaacggctaaagaccaaacagatagtcctgctgatacataaagcaagccagcacctgaagctacgagccatccaacattgctatctcggcttgcaagaagtatggttagtgctgtcatctgcgtggcggttttccacttgcccaagttatttacagcaactgcctctaaaagctttccattttgagatgcagcccattctcttactgcggacatagtaatctccctaccaatgattgcaatagaaggtacggtcaataaccatggaagtggtcctaattcagcaacttggataggttttgtacacagtaaaatcaatgtagctgcaaccataagcttatcagcaactggatccaaaaaggcaccaaacgcagaacctaacctcatcttgcgggcaagatagccgtcaagccagtctgtaatggctgctgcaatgaaaatgcttgttgtagcagttgttccccaccaactatcaacgtaaaaggttgcgacgagaagcgggacggcggcgacacgaccaagtgttaatacggtaggcaatgtaagaactttggaagatgattgcgacggaggcggtgaagaattatcatcactatcaagctgaccgtgaccactgaaactgtttcgggaagaggaagttggtctgctttgctccgacgaagaggatgaagaaaagtaggatagacggtgttggtggcgagatatttgaatcggaaaccttagagatgtacgggaggagtacatgttttcttgccccctatttgcatgaaaatacaatagatgaatagtcattcgctataaaattatttatttgaatatcttatttcctatcagactaagcatagaaatccaatcactaggattattaactaataaggattgtgagtattgaaaaaaagttctgaatctgggggaacacttcactatatattaatatgttggaaccccctttatattatttaaaataatataatttttaataaagggcggcttctcctatgtcggagctcgctcccccgccgtcgttcaatgtgaatggataagaggctcgtgggattgacgtgagggggcagggatggctatatttctgggagaattaaccgatcgacgtgcaagcggacatttattttaaattcgataatttttgcaaaaacatttcgacatatttatttattttattattatgacatgtttttttggggtacagtctatgcctcgggcatccaagcagcaagcgcgttacgccgtgggtcgatgtttgatgttatggagcagcaacgatgttacgcagcagggcagtcgccctaaaacaaagttaaacatcatgggggaagcggtgatcgccgaagtatcgactcaactatcagaggtagttggcgtcatcgagcgccatctcgaaccgacgttgctggccgtacatttgtacggctccgcagtggatggcggcctgaagccacacagtgatattgatttgctggttacggtgaccgtaaggcttgatgaaacaacgcggcgagctttgatcaacgaccttttggaaacttcggcttcccctggagagagcgagattctccgcgctgtagaagtcaccattgttgtgcacgacgacatcattccgtggcgttatccagctaagcgcgaactgcaatttggagaatggcagcgcaatgacattcttgcaggtatcttcgagccagccacgatcgacattgatctggctatcttgctgacaaaagcaagagaacatagcgttgccttggtaggtccagcggcggaggaactctttgatccggttcctgaacaggatctatttgaggcgctaaatgaaaccttaacgctatggaactcgccgcccgactgggctggcgatgagcgaaatgtagtgcttacgttgtcccgcatttggtacagcgcagtaaccggcaaaatcgcgccgaaggatgtcgctgccgactgggcaatggagcgcctgccggcccagtatcagcccgtcatacttgaagctagacaggcttatcttggacaagaagaagatcgcttggcctcgcgcgcagatcagttggaagaatttgtccactacgtgaaaggcgagatcaccaaggtagtcggcaaataaacccaaataatgttttaaaattttaaaaataatgtaggaggaaaaattatggtgagtaaaggtgaagagttgattaaagagaacatgcatatgaagttatacatggagggaactgtcaataatcaccactttaaggctacatcagagggtgagggaaagccatacgagggaacccaaactatgagaatcaaagtagtggagggaggtcctcttccatttgcttttgatatactagcaacaagtttcatgtatggttccaggaccttcattaagcatactcagggaatccctgacttctttaaacagtcttttcctgaaggttttacatgggagagggttaccacttacgaggacggtggagtcttgacagcaacccaggacacttcattacaagatggaatgctaatatacaatgtgaaaattaggggtgtgaatttccctagtaacggaccagttatgcagaagaaaacactaggttgggaagctaatactgaaatgttgtaccctgccgacggaggtttagaaggtagaactgacatggcccttaagctagtcggaggtggacacttgatcgttaactttaaaaccacatataggtctaagaagccagcaaagaatctaaaaatgcctggtgtttactatgtggaccatagactagaaaggataaaagaagcagacaaagaaacttacgtggagcaacatgaggtcgccgtcgctaggtattctgacttaccttccaagctaggtcacaaattgaactccggactctagggatccaaacagtagacattagcagataaattagcaggaaataaagaaggataaggagaaagaactcaagtaattatccttcgttctcttaattgaattgcaattaaactcggcccaatcttttactaaaaggattgagccgaatacaacaaagattctattgcatatattttgactaagtatatacttacctagatatacaagatttgaaatacaaaatctagagcatgcctccacttggctcgggggatatagctcagttggtagagctccgctcttgcaattgggtcgttgcgattacgggttgggtgtctaattgtccaggcggtaatgatagtatcttgtacctgaaccggtggctcactttttctaagtaatggggaaaaggaccgaaacatgccactgaaagactctactgagacaaagatgggctgtcaagaacgtagaggaggtaggatggtcagttggtcagatctagtatggatcgtacatggacggtagttggagtcggcggctctcctagggttccctcgtctgggattgatccctggggaagaggatcaagttggcccttgcgaacagcttgatgcactatctcccttcaaccctttgagcgaaatgcggcaaaaggaaggaaaatccatggaccgaccccatcgtctccaccccgtaggaactacgagatcaccccaaggacgccttcggtatccaggggtcgcggaccgaccatagaaccctgttcaataagtggaatgcattagctgtccgctcgcaggttgggcagtaagggtcggagaagggcaatcactcattcttaaaaccagcattcgaaagagttggggcggaaaagggggggaaagctctccgttcctggttctcctgtagctggatcctctagaaccacaagaatccttagttggaatgggattccagctcatcaccttttgagattttgagaagagttgctctttggagagcacagtacgatgaaagttgtaagctgtgttcgggggggagttcttgtctatcgttggcctctatggtagaatcagtcaggggcctgataggcggtggtttaccctgtggcggatgtcagcggttcgagtccgcttatctccaactcgtgaacttagccgatacaaagctatatgatagcacccaatttttccgattcggcagttcgatctatgatttttcattcatggacgttgataagatctttccatttagcagcaccttaggatggcatagccttaaagttaagggcgaggttcaaacgaggaaaggcttacggtggatacctaggcacccagagacgaggaagggcgtagtaagcgacgaaatgcttcggggagttgaaaataagcgtagatccggagattcccgaataggttaaccttttgaactgctgctgaatccatgggcaggcaagagacaacctggcgaactgaaacatcttagtagccagaggaaaagaaagcaaaagcgattcccgtagtagcggcgagcgaaatgggagcagcctaaaccgtgaaaacggggttgtgggagagcaaaaaaagcgtcgtgctgctaggcgaagcggtggagtgccgcaccctagatggcgagagtccagtagccgaaagcatcactagcttatgctctgacccgagtagcatggggcacgtggaatcccgtgtgaatcagcaaggaccaccttgcaaggctaaatactcctgggtgaccgatagcgaagtagtaccgtgagggaagggtgaaaagaacccccatcggggagtgaaatagaacatgaaaccgtaagctcccaagcagtgggaggagccctgggctctgaccgcgtgcctgttgaagaatgagccggcgactcataggcagtggcttggttaacccagctttcttgtacaaagttggcattataagaaagcattgcttatcaatttgttgcaacgaacaggtcactatcagtcaaaataaaatcattatttgccatccagctgatatcccctatagtgagtcgtattacatggtcatagctgtttcctggcagctctggcccgtgtctcaaaatctctgatgttacattgcacaagataaaaatatatcatcatgaacaataaaactgtctgcttacataaacagtaatacaaggggtgttatgagccatattcaacgggaaacgtcgaggccgcgattaaattccaacatggatgctgatttatatgggtataaatgggctcgcgataatgtcgggcaatcaggtgcgacaatctatcgcttgtatgggaagcccgatgcgccagagttgtttctgaaacatggcaaaggtagcgttgccaatgatgttacagatgagatggtcagactaaactggctgacggaatttatgcctcttccgaccatcaagcattttatccgtactcctgatgatgcatggttactcaccactgcgatccccggaaaaacagcattccaggtattagaagaatatcctgattcaggtgaaaatattgttgatgcgctggcagtgttcctgcgccggttgcattcgattcctgtttgtaattgtccttttaacagcgatcgcgtatttcgtctcgctcaggcgcaatcacgaatgaataacggtttggttgatgcgagtgattttgatgacgagcgtaatggctggcctgttgaacaagtctggaaagaaatgcataaacttttgccattctcaccggattcagtcgtcactcatggtgatttctcacttgataaccttatttttgacgaggggaaattaataggttgtattgatgttggacgagtcggaatcgcagaccgataccaggatcttgccatcctatggaactgcctcggtgagttttctccttcattacagaaacggctttttcaaaaatatggtattgataatcctgatatgaataaattgcagtttcatttgatgctcgatgagtttttctaatcagaattggttaattggttgtaacactggcagagcattacgctgacttgacgggacggcgcaagctcatgaccaaaatcccttaacgtgagttacgcgtcgttccactgagcgtcagaccccgtagaaaagatcaaaggatcttcttgagatcctttttttctgcgcgtaatctgctgcttgcaaacaaaaaaaccaccgctaccagcggtggtttgtttgccggatcaagagctaccaactctttttccgaaggtaactggcttcagcagagcgcagataccaaatactgttcttctagtgtagccgtagttaggccaccacttcaagaactctgtagcaccgcctacatacctcgctctgctaatcctgttaccagtggctgctgccagtggcgataagtcgtgtcttaccgggttggactcaagacgatagttaccggataaggcgcagcggtcgggctgaacggggggttcgtgcacacagcccagcttggagcgaacgacctacaccgaactgagatacctacagcgtgagctatgagaaagcgccacgcttcccgaagggagaaaggcggacaggtatccggtaagcggcagggtcggaacaggagagcgcacgagggagcttccagggggaaacgcctggtatctttatagtcctgtcgggtttcgccacctctgacttgagcgtcgatttttgtgatgctcgtcaggggggcggagcctatggaaaaacgccagcaacgcggcctttttacggttcctggccttttgctggccttttgctcacatgtt

SEQ ID NO: 16 - DNA, 22 bp, Artificial Sequence
  PCR Primer
atgtactcctcccgtacatctc

SEQ ID NO: 17 - DNA, 28 bp, Artificial Sequence
  PCR Primer
ctacttcattagtactttccatatcttc